European Patent Application EP 4 786 594 A1, published August 5, 2026. Title: 用于治疗血红蛋白疾病的组合物和方法. Applicant: 上海天泽云泰生物医药有限公司. The sequence listing filed with the application follows.

SEQUENCE LISTING (92 sequences)

SEQ ID NO: 1 - protein, 1153 aa, synthetic construct
  REGION 1..1153: note = Cas12b-M1
  SITE 1153: note = misc_feature - Xaa =
MHHHHHHPKKKRKVPGAVKSMKVKLRLDNMPEIRAGLWKLHTEVNAGVRYYTEWLSLLRQENLYRRSPNGDGEQECYKTAEECKAELLERLRARQVENGHCGPAGSDDELLQLARQLYELLVPQAIGAKGDAQFIARKFLSPLADKDAVGGLGIAKAGNKPRWVRMREAGEPGWEEEKAKAEARKSTDRTADVLRALADFGLKPLMRVYTDSDMSSVQWKPLRKGQAVRTWDRDMFQQAIERMMSWESWNQRVGEAYAKLVEQKSRFEQKNFVGQEHLVQLVNQLQQDMKEASHGLESKEQTAHYLTGRALRGSDKVFEKWEKLDPDAPFDLYDTEIKNVQRRNTRRFGSHDLFAKLAEPKYQALWREDASFLTRYAVYNSIVRKLNHAKMFATFTLPDATAHPIWTRFDKLGGNLHQYTFLFNEFGEGRHAIRFQKLLTVEDGVAKEVDDVTVPISMSAQLDDLLPRDPHELVALYFQDYGAEQHLAGRFGGAKIQYRRDQLNHLHARRGARDVYLNLSVRVQSQSEARGERRPPYAAVFRLVGDNHRAFVHFDKLSDYLAEHPDDGKLGSEGLLSGLRVMSVDLGLRTSASISVFRVARKDELKPNSEGRVPFCFPIEGNENLVAVHERSQLLKLPGETESKDLRAIREERQRTLRQLRTQLAYLRLLVRCGSEDVGRRERSWAKLIEQPMDANQMTPDWREAFEDELQKLKSLYGICGDREWTEAVYESVRRVWRHGKQVRDWRKDVRSGERPKIRGYQKDVVGGNSIRQIEYLERQYKFLKSWSFFGKVSGQVIRAEKGSRFAITLREHIDHAKEDRLKKLADRIIMEALGYVYALDDERGKGKWVAKYPPCQLILLEELSEYQFNNDRPPSENNQLMQWSHRGVFQELLNQAQVHDLLVGTMYAAFSSRFDARTGAPGIRCRRVPARCAREQNPEPFPWWLNKFVAEHKLDGCPLRADDLIPTGEGEFFVSPFSAEEGDFHQIHADLNAAQNLQRRLWSDFDISQIRLRCDWGEVDGEPVLIPRTTGKRTADSYGNKVFYTKTGVTYYERERGKKRRKVFAQEELSEEEAELLVEADEAREKSVVLMRDPSGIINRGDWTRQKEFWSMVNQRIEGYLVKQIRSRVRLQESACENTGDIASPKKKRKVX

SEQ ID NO: 2 - protein, 1147 aa, synthetic construct
  REGION 1..1147: note = Cas12b-M2
  SITE 1147: note = misc_feature - Xaa =
MPKKKRKVPGAVKSMKVKLRLDNMPEIRAGLWKLHTEVNAGVRYYTEWLSLLRQENLYRRSPNGDGEQECYKTAEECKAELLERLRARQVENGHCGPAGSDDELLQLARQLYELLVPQAIGAKGDAQFIARKFLSPLADKDAVGGLGIAKAGNKPRWVRMREAGEPGWEEEKAKAEARKSTDRTADVLRALADFGLKPLMRVYTDSDMSSVQWKPLRKGQAVRTWDRDMFQQAIERMMSWESWNQRVGEAYAKLVEQKSRFEQKNFVGQEHLVQLVNQLQQDMKEASHGLESKEQTAHYLTGRALRGSDKVFEKWEKLDPDAPFDLYDTEIKNVQRRNTRRFGSHDLFAKLAEPKYQALWREDASFLTRYAVYNSIVRKLNHAKMFATFTLPDATAHPIWTRFDKLGGNLHQYTFLFNEFGEGRHAIRFQKLLTVEDGVAKEVDDVTVPISMSAQLDDLLPRDPHELVALYFQDYGAEQHLAGRFGGAKIQYRRDQLNHLHARRGARDVYLNLSVRVQSQSEARGERRPPYAAVFRLVGDNHRAFVHFDKLSDYLAEHPDDGKLGSEGLLSGLRVMSVDLGLRTSASISVFRVARKDELKPNSEGRVPFCFPIEGNENLVAVHERSQLLKLPGETESKDLRAIREERQRTLRQLRTQLAYLRLLVRCGSEDVGRRERSWAKLIEQPMDANQMTPDWREAFEDELQKLKSLYGICGDREWTEAVYESVRRVWRHGKQVRDWRKDVRSGERPKIRGYQKDVVGGNSIRQIEYLERQYKFLKSWSFFGKVSGQVIRAEKGSRFAITLREHIDHAKEDRLKKLADRIIMEALGYVYALDDERGKGKWVAKYPPCQLILLEELSEYQFNNDRPPSENNQLMQWSHRGVFQELLNQAQVHDLLVGTMYAAFSSRFDARTGAPGIRCRRVPARCAREQNPEPFPWWLNKFVAEHKLDGCPLRADDLIPTGEGEFFVSPFSAEEGDFHQIHADLNAAQNLQRRLWSDFDISQIRLRCDWGEVDGEPVLIPRTTGKRTADSYGNKVFYTKTGVTYYERERGKKRRKVFAQEELSEEEAELLVEADEAREKSVVLMRDPSGIINRGDWTRQKEFWSMVNQRIEGYLVKQIRSRVRLQESACENTGDIASPKKKRKVX

SEQ ID NO: 3 - protein, 1167 aa, synthetic construct
  REGION 1..1167: note = Cas12b-M3
  SITE 1167: note = misc_feature - Xaa =
MPKKKRKVPGAVKSMKVKLRLDNMPEIRAGLWKLHTEVNAGVRYYTEWLSLLRQENLYRRSPNGDGEQECYKTAEECKAELLERLRARQVENGHCGPAGSDDELLQLARQLYELLVPQAIGAKGDAQFIARKFLSPLADKDAVGGLGIAKAGNKPRWVRMREAGEPGWEEEKAKAEARKSTDRTADVLRALADFGLKPLMRVYTDSDMSSVQWKPLRKGQAVRTWDRDMFQQAIERMMSWESWNQRVGEAYAKLVEQKSRFEQKNFVGQEHLVQLVNQLQQDMKEASHGLESKEQTAHYLTGRALRGSDKVFEKWEKLDPDAPFDLYDTEIKNVQRRNTRRFGSHDLFAKLAEPKYQALWREDASFLTRYAVYNSIVRKLNHAKMFATFTLPDATAHPIWTRFDKLGGNLHQYTFLFNEFGEGRHAIRFQKLLTVEDGVAKEVDDVTVPISMSAQLDDLLPRDPHELVALYFQDYGAEQHLAGRFGGAKIQYRRDQLNHLHARRGARDVYLNLSVRVQSQSEARGERRPPYAAVFRLVGDNHRAFVHFDKLSDYLAEHPDDGKLGSEGLLSGLRVMSVDLGLRTSASISVFRVARKDELKPNSEGRVPFCFPIEGNENLVAVHERSQLLKLPGETESKDLRAIREERQRTLRQLRTQLAYLRLLVRCGSEDVGRRERSWAKLIEQPMDANQMTPDWREAFEDELQKLKSLYGICGDREWTEAVYESVRRVWRHGKQVRDWRKDVRSGERPKIRGYQKDVVGGNSIRQIEYLERQYKFLKSWSFFGKVSGQVIRAEKGSRFAITLREHIDHAKEDRLKKLADRIIMEALGYVYALDDERGKGKWVAKYPPCQLILLEELSEYQFNNDRPPSENNQLMQWSHRGVFQELLNQAQVHDLLVGTMYAAFSSRFDARTGAPGIRCRRVPARCAREQNPEPFPWWLNKFVAEHKLDGCPLRADDLIPTGEGEFFVSPFSAEEGDFHQIHADLNAAQNLQRRLWSDFDISQIRLRCDWGEVDGEPVLIPRTTGKRTADSYGNKVFYTKTGVTYYERERGKKRRKVFAQEELSEEEAELLVEADEAREKSVVLMRDPSGIINRGDWTRQKEFWSMVNQRIEGYLVKQIRSRVRLQESACENTGDIASPKKKRKVGSGSKRPAATKKAGQAKKKKX

SEQ ID NO: 4 - protein, 1160 aa, synthetic construct
  REGION 1..1160: note = Cas12b-M4
  SITE 1160: note = misc_feature - Xaa =
MPKKKRKVPGAVKSMKVKLRLDNMPEIRAGLWKLHTEVNAGVRYYTEWLSLLRQENLYRRSPNGDGEQECYKTAEECKAELLERLRARQVENGHCGPAGSDDELLQLARQLYELLVPQAIGAKGDAQFIARKFLSPLADKDAVGGLGIAKAGNKPRWVRMREAGEPGWEEEKAKAEARKSTDRTADVLRALADFGLKPLMRVYTDSDMSSVQWKPLRKGQAVRTWDRDMFQQAIERMMSWESWNQRVGEAYAKLVEQKSRFEQKNFVGQEHLVQLVNQLQQDMKEASHGLESKEQTAHYLTGRALRGSDKVFEKWEKLDPDAPFDLYDTEIKNVQRRNTRRFGSHDLFAKLAEPKYQALWREDASFLTRYAVYNSIVRKLNHAKMFATFTLPDATAHPIWTRFDKLGGNLHQYTFLFNEFGEGRHAIRFQKLLTVEDGVAKEVDDVTVPISMSAQLDDLLPRDPHELVALYFQDYGAEQHLAGRFGGAKIQYRRDQLNHLHARRGARDVYLNLSVRVQSQSEARGERRPPYAAVFRLVGDNHRAFVHFDKLSDYLAEHPDDGKLGSEGLLSGLRVMSVDLGLRTSASISVFRVARKDELKPNSEGRVPFCFPIEGNENLVAVHERSQLLKLPGETESKDLRAIREERQRTLRQLRTQLAYLRLLVRCGSEDVGRRERSWAKLIEQPMDANQMTPDWREAFEDELQKLKSLYGICGDREWTEAVYESVRRVWRHGKQVRDWRKDVRSGERPKIRGYQKDVVGGNSIRQIEYLERQYKFLKSWSFFGKVSGQVIRAEKGSRFAITLREHIDHAKEDRLKKLADRIIMEALGYVYALDDERGKGKWVAKYPPCQLILLEELSEYQFNNDRPPSENNQLMQWSHRGVFQELLNQAQVHDLLVGTMYAAFSSRFDARTGAPGIRCRRVPARCAREQNPEPFPWWLNKFVAEHKLDGCPLRADDLIPTGEGEFFVSPFSAEEGDFHQIHADLNAAQNLQRRLWSDFDISQIRLRCDWGEVDGEPVLIPRTTGKRTADSYGNKVFYTKTGVTYYERERGKKRRKVFAQEELSEEEAELLVEADEAREKSVVLMRDPSGIINRGDWTRQKEFWSMVNQRIEGYLVKQIRSRVRLQESACENTGDIASPKKKRKVGSGSPAAKKKKLDX

SEQ ID NO: 5 - protein, 1180 aa, synthetic construct
  REGION 1..1180: note = Cas12b-M5
  SITE 1180: note = misc_feature - Xaa =
MPAAKKKKLDGSGSPKKKRKVPGAVKSMKVKLRLDNMPEIRAGLWKLHTEVNAGVRYYTEWLSLLRQENLYRRSPNGDGEQECYKTAEECKAELLERLRARQVENGHCGPAGSDDELLQLARQLYELLVPQAIGAKGDAQFIARKFLSPLADKDAVGGLGIAKAGNKPRWVRMREAGEPGWEEEKAKAEARKSTDRTADVLRALADFGLKPLMRVYTDSDMSSVQWKPLRKGQAVRTWDRDMFQQAIERMMSWESWNQRVGEAYAKLVEQKSRFEQKNFVGQEHLVQLVNQLQQDMKEASHGLESKEQTAHYLTGRALRGSDKVFEKWEKLDPDAPFDLYDTEIKNVQRRNTRRFGSHDLFAKLAEPKYQALWREDASFLTRYAVYNSIVRKLNHAKMFATFTLPDATAHPIWTRFDKLGGNLHQYTFLFNEFGEGRHAIRFQKLLTVEDGVAKEVDDVTVPISMSAQLDDLLPRDPHELVALYFQDYGAEQHLAGRFGGAKIQYRRDQLNHLHARRGARDVYLNLSVRVQSQSEARGERRPPYAAVFRLVGDNHRAFVHFDKLSDYLAEHPDDGKLGSEGLLSGLRVMSVDLGLRTSASISVFRVARKDELKPNSEGRVPFCFPIEGNENLVAVHERSQLLKLPGETESKDLRAIREERQRTLRQLRTQLAYLRLLVRCGSEDVGRRERSWAKLIEQPMDANQMTPDWREAFEDELQKLKSLYGICGDREWTEAVYESVRRVWRHGKQVRDWRKDVRSGERPKIRGYQKDVVGGNSIRQIEYLERQYKFLKSWSFFGKVSGQVIRAEKGSRFAITLREHIDHAKEDRLKKLADRIIMEALGYVYALDDERGKGKWVAKYPPCQLILLEELSEYQFNNDRPPSENNQLMQWSHRGVFQELLNQAQVHDLLVGTMYAAFSSRFDARTGAPGIRCRRVPARCAREQNPEPFPWWLNKFVAEHKLDGCPLRADDLIPTGEGEFFVSPFSAEEGDFHQIHADLNAAQNLQRRLWSDFDISQIRLRCDWGEVDGEPVLIPRTTGKRTADSYGNKVFYTKTGVTYYERERGKKRRKVFAQEELSEEEAELLVEADEAREKSVVLMRDPSGIINRGDWTRQKEFWSMVNQRIEGYLVKQIRSRVRLQESACENTGDIASPKKKRKVGSGSKRPAATKKAGQAKKKKX

SEQ ID NO: 6 - protein, 1173 aa, synthetic construct
  REGION 1..1173: note = Cas12b-M6
  SITE 1173: note = misc_feature - Xaa =
MPGAVKSMKVKLRLDNMPEIRAGLWKLHTEVNAGVRYYTEWLSLLRQENLYRRSPNGDGEQECYKTAEECKAELLERLRARQVENGHCGPAGSDDELLQLARQLYELLVPQAIGAKGDAQFIARKFLSPLADKDAVGGLGIAKAGNKPRWVRMREAGEPGWEEEKAKAEARKSTDRTADVLRALADFGLKPLMRVYTDSDMSSVQWKPLRKGQAVRTWDRDMFQQAIERMMSWESWNQRVGEAYAKLVEQKSRFEQKNFVGQEHLVQLVNQLQQDMKEASHGLESKEQTAHYLTGRALRGSDKVFEKWEKLDPDAPFDLYDTEIKNVQRRNTRRFGSHDLFAKLAEPKYQALWREDASFLTRYAVYNSIVRKLNHAKMFATFTLPDATAHPIWTRFDKLGGNLHQYTFLFNEFGEGRHAIRFQKLLTVEDGVAKEVDDVTVPISMSAQLDDLLPRDPHELVALYFQDYGAEQHLAGRFGGAKIQYRRDQLNHLHARRGARDVYLNLSVRVQSQSEARGERRPPYAAVFRLVGDNHRAFVHFDKLSDYLAEHPDDGKLGSEGLLSGLRVMSVDLGLRTSASISVFRVARKDELKPNSEGRVPFCFPIEGNENLVAVHERSQLLKLPGETESKDLRAIREERQRTLRQLRTQLAYLRLLVRCGSEDVGRRERSWAKLIEQPMDANQMTPDWREAFEDELQKLKSLYGICGDREWTEAVYESVRRVWRHGKQVRDWRKDVRSGERPKIRGYQKDVVGGNSIRQIEYLERQYKFLKSWSFFGKVSGQVIRAEKGSRFAITLREHIDHAKEDRLKKLADRIIMEALGYVYALDDERGKGKWVAKYPPCQLILLEELSEYQFNNDRPPSENNQLMQWSHRGVFQELLNQAQVHDLLVGTMYAAFSSRFDARTGAPGIRCRRVPARCAREQNPEPFPWWLNKFVAEHKLDGCPLRADDLIPTGEGEFFVSPFSAEEGDFHQIHADLNAAQNLQRRLWSDFDISQIRLRCDWGEVDGEPVLIPRTTGKRTADSYGNKVFYTKTGVTYYERERGKKRRKVFAQEELSEEEAELLVEADEAREKSVVLMRDPSGIINRGDWTRQKEFWSMVNQRIEGYLVKQIRSRVRLQESACENTGDIASPKKKRKVGSGSPAAKKKKLDGSGSKRPAATKKAGQAKKKKX

SEQ ID NO: 7 - protein, 1171 aa, synthetic construct
  REGION 1..1171: note = Cas12b-M7
  SITE 1171: note = misc_feature - Xaa =
MKRTADGSEFESPKKKRKVEPGAVKSMKVKLRLDNMPEIRAGLWKLHTEVNAGVRYYTEWLSLLRQENLYRRSPNGDGEQECYKTAEECKAELLERLRARQVENGHCGPAGSDDELLQLARQLYELLVPQAIGAKGDAQFIARKFLSPLADKDAVGGLGIAKAGNKPRWVRMREAGEPGWEEEKAKAEARKSTDRTADVLRALADFGLKPLMRVYTDSDMSSVQWKPLRKGQAVRTWDRDMFQQAIERMMSWESWNQRVGEAYAKLVEQKSRFEQKNFVGQEHLVQLVNQLQQDMKEASHGLESKEQTAHYLTGRALRGSDKVFEKWEKLDPDAPFDLYDTEIKNVQRRNTRRFGSHDLFAKLAEPKYQALWREDASFLTRYAVYNSIVRKLNHAKMFATFTLPDATAHPIWTRFDKLGGNLHQYTFLFNEFGEGRHAIRFQKLLTVEDGVAKEVDDVTVPISMSAQLDDLLPRDPHELVALYFQDYGAEQHLAGRFGGAKIQYRRDQLNHLHARRGARDVYLNLSVRVQSQSEARGERRPPYAAVFRLVGDNHRAFVHFDKLSDYLAEHPDDGKLGSEGLLSGLRVMSVDLGLRTSASISVFRVARKDELKPNSEGRVPFCFPIEGNENLVAVHERSQLLKLPGETESKDLRAIREERQRTLRQLRTQLAYLRLLVRCGSEDVGRRERSWAKLIEQPMDANQMTPDWREAFEDELQKLKSLYGICGDREWTEAVYESVRRVWRHGKQVRDWRKDVRSGERPKIRGYQKDVVGGNSIRQIEYLERQYKFLKSWSFFGKVSGQVIRAEKGSRFAITLREHIDHAKEDRLKKLADRIIMEALGYVYALDDERGKGKWVAKYPPCQLILLEELSEYQFNNDRPPSENNQLMQWSHRGVFQELLNQAQVHDLLVGTMYAAFSSRFDARTGAPGIRCRRVPARCAREQNPEPFPWWLNKFVAEHKLDGCPLRADDLIPTGEGEFFVSPFSAEEGDFHQIHADLNAAQNLQRRLWSDFDISQIRLRCDWGEVDGEPVLIPRTTGKRTADSYGNKVFYTKTGVTYYERERGKKRRKVFAQEELSEEEAELLVEADEAREKSVVLMRDPSGIINRGDWTRQKEFWSMVNQRIEGYLVKQIRSRVRLQESACENTGDIASKRTADGSEFESPKKKRKVEX

SEQ ID NO: 8 - protein, 1182 aa, synthetic construct
  REGION 1..1182: note = Cas12b-M8
  SITE 1182: note = misc_feature - Xaa =
MPKKKRKVTRMAVKSMKVKLRLDNMPEIRAGLWKLHTEVNAGVRYYTEWLSLLRQENLYRRSPNGDGEQECYKTAEECKAELLERLRARQVENGHCGPAGSDDELLQLARQLYELLVPQAIGAKGDAQFIARKFLSPLADKDAVGGLGIAKAGNKPRWVRMREAGEPGWEEEKAKAEARKSTDRTADVLRALADFGLKPLMRVYTDSDMSSVQWKPLRKGQAVRTWDRDMFQQAIERMMSWESWNQRVGEAYAKLVEQKSRFEQKNFVGQEHLVQLVNQLQQDMKEASHGLESKEQTAHYLTGRALRGSDKVFEKWEKLDPDAPFDLYDTEIKNVQRRNTRRFGSHDLFAKLAEPKYQALWREDASFLTRYAVYNSIVRKLNHAKMFATFTLPDATAHPIWTRFDKLGGNLHQYTFLFNEFGEGRHAIRFQKLLTVEDGVAKEVDDVTVPISMSAQLDDLLPRDPHELVALYFQDYGAEQHLAGRFGGAKIQYRRDQLNHLHARRGARDVYLNLSVRVQSQSEARGERRPPYAAVFRLVGDNHRAFVHFDKLSDYLAEHPDDGKLGSEGLLSGLRVMSVDLGLRTSASISVFRVARKDELKPNSEGRVPFCFPIEGNENLVAVHERSQLLKLPGETESKDLRAIREERQRTLRQLRTQLAYLRLLVRCGSEDVGRRERSWAKLIEQPMDANQMTPDWREAFEDELQKLKSLYGICGDREWTEAVYESVRRVWRHMGKQVRDWRKDVRSGERPKIRGYQKDVVGGNSIRQIEYLERQYKFLKSWSFFGKVSGQVIRAEKGSRFAITLREHIDHAKEDRLKKLADRIIMEALGYVYALDDERGKGKWVAKYPPCQLILLEELSEYQFNNDRPPSENNQLMQWSHRGVFQELLNQAQVHDLLVGTMYAAFSSRFDARTGAPGIRCRRVPARCAREQNPEPFPWWLNKFVAEHKLDGCPLRADDLIPTGEGEFFVSPFSAEEGDFHQIHADLNAAQNLQRRLWSDFDISQIRLRCDWGEVDGEPVLIPRTTGKRTADSYGNKVFYTKTGVTYYERERGKKRRKVFAQEELSEEEAELLVEADEAREKSVVLMRDPSGIINRGDWTRQKEFWSMVNQRIEGYLVKQIRSRVRLQESACENTGDIASPKKKRKVGSGSPAAKKKKLDGSGSKRPAATKKAGQAKKKKX

SEQ ID NO: 9 - protein, 1080 aa, synthetic construct
  REGION 1..1080: note = Cas12i-M1
  SITE 1080: note = misc_feature - Xaa =
MHHHHHHPKKKRKVPGMSSAIKSYKSVLRPNERKNQLLKSTIQCLEDGSAFFFKMLQGLFGGITPEIVRFSTEQEKQQQDIALWCAVNWFRPVSQDSLTHTIASDNLVEKFEEYYGGTASDAIKQYFSASIGESYYWNDCRQQYYDLCRELGVEVSDLTHDLEILCREKCLAVATESNQYNSIISVLFGTGRKEDRSVKLRITKKILEAISNLKEIPKNVAPIQEIILNVAKATKETFRQVYAGNLGAPSTLERFIAKDGQKEFDLKKLQTDLKKVIRGKSKERDWCCQEELRSYVEQNTIQYDLWAWGEMFNKAHTALKIKSTRNYNFAKQRLEQFKRIQSLNNLLVVKKLNDFFDSEFFSGEETYTICVHHLGGKRLSKLYKAWEDDPADPENAIVVLCDDLKNNFKAEPIRNILRYIFTIRQECSAQDILAAAKYNQQLDRYKSQKANPSVLGNQGFTWRNAVILPEKAQRNDRPNSLDLRIWLYLKLRHPDGRWKKHHIPFYDTRFFQEIYAAGNSPVDTCQFRTPRFGYHLPKLTDQTAIRVNKKHVKAAKTEARIRLAIQQGTLPVSNLKITRISATINSKGQVRIPVKFDVGRQKGTLQIGDRFCGYDQNQTASHAYSLWEVVKEGQYHKELGCFVRFISSGDIVSITENRGNQFDQLSYEGLAYPQYADWRKKASKFVSLWQITKKNKKKEIVTVEAKEKFDAICKYQPRLYKFNKEYAYLLRDIVRGKSLVELQQIRQEIFRFIEQDCGVTRLGSLSLSTLETVKAVKGIIYSYFSTALNASKNNPISDEQRKEFDPELFALLEKLELIRTRKKKQKVERIANSLIQTCLENNIKFIRGEGDLSTTNNATKKKANSRSMDWLARGVFNKIRQLAPMHNITLFGCGSLYTSHQDPLVHRNPDKAMKCRWAAIPVKDIGDWVLRKLSQNLRAKNIGTGEYYHQGVKEFLSHYELQDLEEELLKWRSDRKSNIPCWVLQNRLAEKLGNKEAVVYIPVRGGRIYFATHKVATGAVSIVFDQKQVWVCNADHVAAANIALTVKGIGEQSSDEENPDGSRIKLQLTSASPKKKRKVX

SEQ ID NO: 10 - protein, 1080 aa, synthetic construct
  REGION 1..1080: note = Cas12i-M2
  SITE 1080: note = misc_feature - Xaa =
MHHHHHHPKKKRKVPGMSSAIKSYKSVLRPNERKNQLLKSTIQCLEDGSAFFFKMLQGLFGGITPEIVRFSTEQEKQQQDIALWCAVNWFRPVSQDSLTHTIASDNLVEKFEEYYGGTASDAIKQYFSASIGESYYWNDCRQQYYDLCRELGVEVSDLTHDLEILCREKCLAVATESNQYNSIISVLFGTGRKEDRSVKLRITKKILEAISNLKEIPKNVAPIQEIILNVAKATKETFRQVYAGNLGAPSTLERFIAKDGQKEFDLKKLQTDLKKVIRGKSKERDWCCQEELRSYVEQNTIQYDLWAWGEMFNKAHTALKIKSTRNYNFAKQRLEQFKRIQSLNNLLVVKKLNDFFDSEFFSGEETYTICVHHLGGKRLSKLYKAWEDDPADPENAIVVLCDDLKNNFKKEPIRNILRYIFTIRQECSAQDILAAAKYNQQLDRYKSQKANPSVLGNQGFTWRNAVILPEKAQRNDRPNSLDLRIWLYLKLRHPDGRWKKHHIPFYDTRFFQEIYAAGNSPVDTCQFRTPRFGYHLPKLTDQTAIRVNKKHVKAAKTEARIRLAIQQGTLPVSNLKITRISATINSKGQVRIPVKFDVGRQKGTLQIGDRFCGYDQNQTASHAYSLWEVVKEGQYHKELGCFVRFISSGDIVSITENRGNQFDQLSYEGLAYPQYADWRKKASKFVSLWQITKKNKKKEIVTVEAKEKFDAICKYQPRLYKFNKEYAYLLRDIVRGKSLVELQQIRQEIFRFIEQDCGVTRLGSLSLSTLETVKAVKGIIYSYFSTALNASKNNPISDEQRKEFDPELFALLEKLELIRTRKKKQKVERIANSLIQTCLENNIKFIRGEGDLSTTNNATKKKANSRSMDWLARGVFNKIRQLAPMHNITLFGCGSLYTSHQDPLVHRNPDKAMKCRWAAIPVKDIGDWVLRKLSQNLRAKNIGTGEYYHQGVKEFLSHYELQDLEEELLKWRSDRKSNIPCWVLQNRLAEKLGNKEAVVYIPVRGGRIYFATHKVATGAVSIVFDQKQVWVCNADHVAAANIALTVKGIGEQSSDEENPDGSRIKLQLTSASPKKKRKVX

SEQ ID NO: 11 - protein, 1072 aa, synthetic construct
  REGION 1..1072: note = Cas12i-M3
PKKKRKVPGMSSAIKSYKSVLRPNERKNQLLKSTIQCLEDGSAFFFKMLQGLFGGITPEIVRFSTEQEKQQQDIALWCAVNWFRPVSQDSLTHTIASDNLVEKFEEYYGGTASDAIKQYFSASIGESYYWNDCRQQYYDLCRELGVEVSDLTHDLEILCREKCLAVATESNQYNSIISVLFGTGRKEDRSVKLRITKKILEAISNLKEIPKNVAPIQEIILNVAKATKETFRQVYAGNLGAPSTLERFIAKDGQKEFDLKKLQTDLKKVIRGKSKERDWCCQEELRSYVEQNTIQYDLWAWGEMFNKAHTALKIKSTRNYNFAKQRLEQFKRIQSLNNLLVVKKLNDFFDSEFFSGEETYTICVHHLGGKRLSKLYKAWEDDPADPENAIVVLCDDLKNNFKKEPIRNILRYIFTIRQECSAQDILAAAKYNQQLDRYKSQKANPSVLGNQGFTWRNAVILPEKAQRNDRPNSLDLRIWLYLKLRHPDGRWKKHHIPFYDTRFFQEIYAAGNSPVDTCQFRTPRFGYHLPKLTDQTAIRVNKKHVKAAKTEARIRLAIQQGTLPVSNLKITRISATINSKGQVRIPVKFDVGRQKGTLQIGDRFCGYDQNQTASHAYSLWEVVKEGQYHKELGCFVRFISSGDIVSITENRGNQFDQLSYEGLAYPQYADWRKKASKFVSLWQITKKNKKKEIVTVEAKEKFDAICKYQPRLYKFNKEYAYLLRDIVRGKSLVELQQIRQEIFRFIEQDCGVTRLGSLSLSTLETVKAVKGIIYSYFSTALNASKNNPISDEQRKEFDPELFALLEKLELIRTRKKKQKVERIANSLIQTCLENNIKFIRGEGDLSTTNNATKKKANSRSMDWLARGVFNKIRQLAPMHNITLFGCGSLYTSHQDPLVHRNPDKAMKCRWAAIPVKDIGDWVLRKLSQNLRAKNIGTGEYYHQGVKEFLSHYELQDLEEELLKWRSDRKSNIPCWVLQNRLAEKLGNKEAVVYIPVRGGRIYFATHKVATGAVSIVFDQKQVWVCNADHVAAANIALTVKGIGEQSSDEENPDGSRIKLQLTSASPKKKRKV

SEQ ID NO: 12 - DNA, 111 bp, synthetic construct
  misc_feature 1..111: note = 12b-gRNA1-18
  source 1..111: mol_type = other DNA
  modified_base 1..3: mod_base = OTHER; note = 2'-O-methyl nucleotide
  modified_base 1..4: mod_base = OTHER; note = phosphorothioate internucleotide linkage
  modified_base 109..111: mod_base = OTHER; note = 2'-O-methyl nucleotide
  modified_base 108..111: mod_base = OTHER; note = phosphorothioate internucleotide linkage
gcaggtcgtctataggacggcgagtttttcaacgggtgtgccaatggccactttccaggtggcaaagcccgttgagcttcaaagaagtggcacagatagtgtggggaaggg

SEQ ID NO: 13 - DNA, 113 bp, synthetic construct
  misc_feature 1..113: note = 12b-gRNA1-20
  source 1..113: mol_type = other DNA
  modified_base 1..3: mod_base = OTHER; note = 2'-O-methyl nucleotide
  modified_base 1..4: mod_base = OTHER; note = phosphorothioate internucleotide linkage
  modified_base 111..113: mod_base = OTHER; note = 2'-O-methyl nucleotide
  modified_base 110..113: mod_base = OTHER; note = phosphorothioate internucleotide linkage
gcaggtcgtctataggacggcgagtttttcaacgggtgtgccaatggccactttccaggtggcaaagcccgttgagcttcaaagaagtggcacagatagtgtggggaaggggc

SEQ ID NO: 14 - DNA, 114 bp, synthetic construct
  misc_feature 1..114: note = 12b-gRNA1-21
  source 1..114: mol_type = other DNA
  modified_base 1..3: mod_base = OTHER; note = 2'-O-methyl nucleotide
  modified_base 1..4: mod_base = OTHER; note = phosphorothioate internucleotide linkage
  modified_base 112..114: mod_base = OTHER; note = 2'-O-methyl nucleotide
  modified_base 111..114: mod_base = OTHER; note = phosphorothioate internucleotide linkage
gcaggtcgtctataggacggcgagtttttcaacgggtgtgccaatggccactttccaggtggcaaagcccgttgagcttcaaagaagtggcacagatagtgtggggaaggggcc

SEQ ID NO: 15 - DNA, 115 bp, synthetic construct
  misc_feature 1..115: note = 12b-gRNA1-22
  source 1..115: mol_type = other DNA
  modified_base 1..3: mod_base = OTHER; note = 2'-O-methyl nucleotide
  modified_base 1..4: mod_base = OTHER; note = phosphorothioate internucleotide linkage
  modified_base 113..115: mod_base = OTHER; note = 2'-O-methyl nucleotide
  modified_base 112..115: mod_base = OTHER; note = phosphorothioate internucleotide linkage
gcaggtcgtctataggacggcgagtttttcaacgggtgtgccaatggccactttccaggtggcaaagcccgttgagcttcaaagaagtggcacagatagtgtggggaaggggccc

SEQ ID NO: 16 - DNA, 116 bp, synthetic construct
  misc_feature 1..116: note = 12b-gRNA1-23
  source 1..116: mol_type = other DNA
  modified_base 1..3: mod_base = OTHER; note = 2'-O-methyl nucleotide
  modified_base 1..4: mod_base = OTHER; note = phosphorothioate internucleotide linkage
  modified_base 114..116: mod_base = OTHER; note = 2'-O-methyl nucleotide
  modified_base 113..116: mod_base = OTHER; note = phosphorothioate internucleotide linkage
gcaggtcgtctataggacggcgagtttttcaacgggtgtgccaatggccactttccaggtggcaaagcccgttgagcttcaaagaagtggcacagatagtgtggggaaggggcccc

SEQ ID NO: 17 - DNA, 117 bp, synthetic construct
  misc_feature 1..117: note = 12b-gRNA1-24
  source 1..117: mol_type = other DNA
  modified_base 1..3: mod_base = OTHER; note = 2'-O-methyl nucleotide
  modified_base 1..4: mod_base = OTHER; note = phosphorothioate internucleotide linkage
  modified_base 115..117: mod_base = OTHER; note = 2'-O-methyl nucleotide
  modified_base 114..117: mod_base = OTHER; note = phosphorothioate internucleotide linkage
gcaggtcgtctataggacggcgagtttttcaacgggtgtgccaatggccactttccaggtggcaaagcccgttgagcttcaaagaagtggcacagatagtgtggggaaggggccccc

SEQ ID NO: 18 - DNA, 118 bp, synthetic construct
  misc_feature 1..118: note = 12b-gRNA1-25
  source 1..118: mol_type = other DNA
  modified_base 1..3: mod_base = OTHER; note = 2'-O-methyl nucleotide
  modified_base 1..4: mod_base = OTHER; note = phosphorothioate internucleotide linkage
  modified_base 116..118: mod_base = OTHER; note = 2'-O-methyl nucleotide
  modified_base 115..118: mod_base = OTHER; note = phosphorothioate internucleotide linkage
gcaggtcgtctataggacggcgagtttttcaacgggtgtgccaatggccactttccaggtggcaaagcccgttgagcttcaaagaagtggcacagatagtgtggggaaggggccccca

SEQ ID NO: 19 - DNA, 119 bp, synthetic construct
  misc_feature 1..119: note = 12b-gRNA1-26
  source 1..119: mol_type = other DNA
  modified_base 1..3: mod_base = OTHER; note = 2'-O-methyl nucleotide
  modified_base 1..4: mod_base = OTHER; note = phosphorothioate internucleotide linkage
  modified_base 117..119: mod_base = OTHER; note = 2'-O-methyl nucleotide
  modified_base 116..119: mod_base = OTHER; note = phosphorothioate internucleotide linkage
gcaggtcgtctataggacggcgagtttttcaacgggtgtgccaatggccactttccaggtggcaaagcccgttgagcttcaaagaagtggcacagatagtgtggggaaggggcccccaa

SEQ ID NO: 20 - DNA, 120 bp, synthetic construct
  misc_feature 1..120: note = 12b-gRNA1-27
  source 1..120: mol_type = other DNA
  modified_base 1..3: mod_base = OTHER; note = 2'-O-methyl nucleotide
  modified_base 1..4: mod_base = OTHER; note = phosphorothioate internucleotide linkage
  modified_base 118..120: mod_base = OTHER; note = 2'-O-methyl nucleotide
  modified_base 117..120: mod_base = OTHER; note = phosphorothioate internucleotide linkage
gcaggtcgtctataggacggcgagtttttcaacgggtgtgccaatggccactttccaggtggcaaagcccgttgagcttcaaagaagtggcacagatagtgtggggaaggggcccccaag

SEQ ID NO: 21 - DNA, 121 bp, synthetic construct
  misc_feature 1..121: note = 12b-gRNA1-28
  source 1..121: mol_type = other DNA
  modified_base 1..3: mod_base = OTHER; note = 2'-O-methyl nucleotide
  modified_base 1..4: mod_base = OTHER; note = phosphorothioate internucleotide linkage
  modified_base 119..121: mod_base = OTHER; note = 2'-O-methyl nucleotide
  modified_base 118..121: mod_base = OTHER; note = phosphorothioate internucleotide linkage
gcaggtcgtctataggacggcgagtttttcaacgggtgtgccaatggccactttccaggtggcaaagcccgttgagcttcaaagaagtggcacagatagtgtggggaaggggcccccaaga

SEQ ID NO: 22 - DNA, 122 bp, synthetic construct
  misc_feature 1..122: note = 12b-gRNA1-29
  source 1..122: mol_type = other DNA
  modified_base 1..3: mod_base = OTHER; note = 2'-O-methyl nucleotide
  modified_base 1..4: mod_base = OTHER; note = phosphorothioate internucleotide linkage
  modified_base 120..122: mod_base = OTHER; note = 2'-O-methyl nucleotide
  modified_base 119..122: mod_base = OTHER; note = phosphorothioate internucleotide linkage
gcaggtcgtctataggacggcgagtttttcaacgggtgtgccaatggccactttccaggtggcaaagcccgttgagcttcaaagaagtggcacagatagtgtggggaaggggcccccaagag

SEQ ID NO: 23 - DNA, 123 bp, synthetic construct
  misc_feature 1..123: note = 12b-gRNA1-30
  source 1..123: mol_type = other DNA
  modified_base 1..3: mod_base = OTHER; note = 2'-O-methyl nucleotide
  modified_base 1..4: mod_base = OTHER; note = phosphorothioate internucleotide linkage
  modified_base 121..123: mod_base = OTHER; note = 2'-O-methyl nucleotide
  modified_base 120..123: mod_base = OTHER; note = phosphorothioate internucleotide linkage
gcaggtcgtctataggacggcgagtttttcaacgggtgtgccaatggccactttccaggtggcaaagcccgttgagcttcaaagaagtggcacagatagtgtggggaaggggcccccaagagg

SEQ ID NO: 24 - DNA, 124 bp, synthetic construct
  misc_feature 1..124: note = 12b-gRNA1-31
  source 1..124: mol_type = other DNA
  modified_base 1..3: mod_base = OTHER; note = 2'-O-methyl nucleotide
  modified_base 1..4: mod_base = OTHER; note = phosphorothioate internucleotide linkage
  modified_base 122..124: mod_base = OTHER; note = 2'-O-methyl nucleotide
  modified_base 121..124: mod_base = OTHER; note = phosphorothioate internucleotide linkage
gcaggtcgtctataggacggcgagtttttcaacgggtgtgccaatggccactttccaggtggcaaagcccgttgagcttcaaagaagtggcacagatagtgtggggaaggggcccccaagagga

SEQ ID NO: 25 - DNA, 111 bp, synthetic construct
  misc_feature 1..111: note = 12b-gRNA2-18
  source 1..111: mol_type = other DNA
  modified_base 1..3: mod_base = OTHER; note = 2'-O-methyl nucleotide
  modified_base 1..4: mod_base = OTHER; note = phosphorothioate internucleotide linkage
  modified_base 109..111: mod_base = OTHER; note = 2'-O-methyl nucleotide
  modified_base 108..111: mod_base = OTHER; note = phosphorothioate internucleotide linkage
gcaggtcgtctataggacggcgagtttttcaacgggtgtgccaatggccactttccaggtggcaaagcccgttgagcttcaaagaagtggcaccattgagatagtgtgggg

SEQ ID NO: 26 - DNA, 113 bp, synthetic construct
  misc_feature 1..113: note = 12b-gRNA2-20
  source 1..113: mol_type = other DNA
  modified_base 1..3: mod_base = OTHER; note = 2'-O-methyl nucleotide
  modified_base 1..4: mod_base = OTHER; note = phosphorothioate internucleotide linkage
  modified_base 111..113: mod_base = OTHER; note = 2'-O-methyl nucleotide
  modified_base 110..113: mod_base = OTHER; note = phosphorothioate internucleotide linkage
gcaggtcgtctataggacggcgagtttttcaacgggtgtgccaatggccactttccaggtggcaaagcccgttgagcttcaaagaagtggcaccattgagatagtgtggggaa

SEQ ID NO: 27 - DNA, 114 bp, synthetic construct
  misc_feature 1..114: note = 12b-gRNA2-21
  source 1..114: mol_type = other DNA
  modified_base 1..3: mod_base = OTHER; note = 2'-O-methyl nucleotide
  modified_base 1..4: mod_base = OTHER; note = phosphorothioate internucleotide linkage
  modified_base 112..114: mod_base = OTHER; note = 2'-O-methyl nucleotide
  modified_base 111..114: mod_base = OTHER; note = phosphorothioate internucleotide linkage
gcaggtcgtctataggacggcgagtttttcaacgggtgtgccaatggccactttccaggtggcaaagcccgttgagcttcaaagaagtggcaccattgagatagtgtggggaag

SEQ ID NO: 28 - DNA, 115 bp, synthetic construct
  misc_feature 1..115: note = 12b-gRNA2-22
  source 1..115: mol_type = other DNA
  modified_base 1..3: mod_base = OTHER; note = 2'-O-methyl nucleotide
  modified_base 1..4: mod_base = OTHER; note = phosphorothioate internucleotide linkage
  modified_base 113..115: mod_base = OTHER; note = 2'-O-methyl nucleotide
  modified_base 112..115: mod_base = OTHER; note = phosphorothioate internucleotide linkage
gcaggtcgtctataggacggcgagtttttcaacgggtgtgccaatggccactttccaggtggcaaagcccgttgagcttcaaagaagtggcaccattgagatagtgtggggaagg

SEQ ID NO: 29 - DNA, 116 bp, synthetic construct
  misc_feature 1..116: note = 12b-gRNA2-23
  source 1..116: mol_type = other DNA
  modified_base 1..3: mod_base = OTHER; note = 2'-O-methyl nucleotide
  modified_base 1..4: mod_base = OTHER; note = phosphorothioate internucleotide linkage
  modified_base 114..116: mod_base = OTHER; note = 2'-O-methyl nucleotide
  modified_base 113..116: mod_base = OTHER; note = phosphorothioate internucleotide linkage
gcaggtcgtctataggacggcgagtttttcaacgggtgtgccaatggccactttccaggtggcaaagcccgttgagcttcaaagaagtggcaccattgagatagtgtggggaaggg

SEQ ID NO: 30 - DNA, 117 bp, synthetic construct
  misc_feature 1..117: note = 12b-gRNA2-24
  source 1..117: mol_type = other DNA
  modified_base 1..3: mod_base = OTHER; note = 2'-O-methyl nucleotide
  modified_base 1..4: mod_base = OTHER; note = phosphorothioate internucleotide linkage
  modified_base 115..117: mod_base = OTHER; note = 2'-O-methyl nucleotide
  modified_base 114..117: mod_base = OTHER; note = phosphorothioate internucleotide linkage
gcaggtcgtctataggacggcgagtttttcaacgggtgtgccaatggccactttccaggtggcaaagcccgttgagcttcaaagaagtggcaccattgagatagtgtggggaagggg

SEQ ID NO: 31 - DNA, 118 bp, synthetic construct
  misc_feature 1..118: note = 12b-gRNA2-25
  source 1..118: mol_type = other DNA
  modified_base 1..3: mod_base = OTHER; note = 2'-O-methyl nucleotide
  modified_base 1..4: mod_base = OTHER; note = phosphorothioate internucleotide linkage
  modified_base 116..118: mod_base = OTHER; note = 2'-O-methyl nucleotide
  modified_base 115..118: mod_base = OTHER; note = 2'-O-methyl nucleotide
gcaggtcgtctataggacggcgagtttttcaacgggtgtgccaatggccactttccaggtggcaaagcccgttgagcttcaaagaagtggcaccattgagatagtgtggggaaggggc

SEQ ID NO: 32 - DNA, 119 bp, synthetic construct
  misc_feature 1..119: note = 12b-gRNA2-26
  source 1..119: mol_type = other DNA
  modified_base 1..3: mod_base = OTHER; note = 2'-O-methyl nucleotide
  modified_base 1..4: mod_base = OTHER; note = phosphorothioate internucleotide linkage
  modified_base 117..119: mod_base = OTHER; note = 2'-O-methyl nucleotide
  modified_base 116..119: mod_base = OTHER; note = phosphorothioate internucleotide linkage
gcaggtcgtctataggacggcgagtttttcaacgggtgtgccaatggccactttccaggtggcaaagcccgttgagcttcaaagaagtggcaccattgagatagtgtggggaaggggcc

SEQ ID NO: 33 - DNA, 120 bp, synthetic construct
  misc_feature 1..120: note = 12b-gRNA2-27
  source 1..120: mol_type = other DNA
  modified_base 1..3: mod_base = OTHER; note = 2'-O-methyl nucleotide
  modified_base 1..4: mod_base = OTHER; note = phosphorothioate internucleotide linkage
  modified_base 118..120: mod_base = OTHER; note = 2'-O-methyl nucleotide
  modified_base 117..120: mod_base = OTHER; note = phosphorothioate internucleotide linkage
gcaggtcgtctataggacggcgagtttttcaacgggtgtgccaatggccactttccaggtggcaaagcccgttgagcttcaaagaagtggcaccattgagatagtgtggggaaggggccc

SEQ ID NO: 34 - DNA, 121 bp, synthetic construct
  misc_feature 1..121: note = 12b-gRNA2-28
  source 1..121: mol_type = other DNA
  modified_base 1..3: mod_base = OTHER; note = 2'-O-methyl nucleotide
  modified_base 1..4: mod_base = OTHER; note = phosphorothioate internucleotide linkage
  modified_base 119..121: mod_base = OTHER; note = 2'-O-methyl nucleotide
  modified_base 118..121: mod_base = OTHER; note = phosphorothioate internucleotide linkage
gcaggtcgtctataggacggcgagtttttcaacgggtgtgccaatggccactttccaggtggcaaagcccgttgagcttcaaagaagtggcaccattgagatagtgtggggaaggggcccc

SEQ ID NO: 35 - DNA, 122 bp, synthetic construct
  misc_feature 1..122: note = 12b-gRNA2-29
  source 1..122: mol_type = other DNA
  modified_base 1..3: mod_base = OTHER; note = 2'-O-methyl nucleotide
  modified_base 1..4: mod_base = OTHER; note = phosphorothioate internucleotide linkage
  modified_base 120..122: mod_base = OTHER; note = 2'-O-methyl nucleotide
  modified_base 119..122: mod_base = OTHER; note = phosphorothioate internucleotide linkage
gcaggtcgtctataggacggcgagtttttcaacgggtgtgccaatggccactttccaggtggcaaagcccgttgagcttcaaagaagtggcaccattgagatagtgtggggaaggggccccc

SEQ ID NO: 36 - DNA, 123 bp, synthetic construct
  misc_feature 1..123: note = 12b-gRNA2-30
  source 1..123: mol_type = other DNA
  modified_base 1..3: mod_base = OTHER; note = 2'-O-methyl nucleotide
  modified_base 1..4: mod_base = OTHER; note = phosphorothioate internucleotide linkage
  modified_base 121..123: mod_base = OTHER; note = 2'-O-methyl nucleotide
  modified_base 120..123: mod_base = OTHER; note = phosphorothioate internucleotide linkage
gcaggtcgtctataggacggcgagtttttcaacgggtgtgccaatggccactttccaggtggcaaagcccgttgagcttcaaagaagtggcaccattgagatagtgtggggaaggggccccca

SEQ ID NO: 37 - DNA, 124 bp, synthetic construct
  misc_feature 1..124: note = 12b-gRNA2-31
  source 1..124: mol_type = other DNA
  modified_base 1..3: mod_base = OTHER; note = 2'-O-methyl nucleotide
  modified_base 1..4: mod_base = OTHER; note = phosphorothioate internucleotide linkage
  modified_base 122..124: mod_base = OTHER; note = 2'-O-methyl nucleotide
  modified_base 121..124: mod_base = OTHER; note = phosphorothioate internucleotide linkage
gcaggtcgtctataggacggcgagtttttcaacgggtgtgccaatggccactttccaggtggcaaagcccgttgagcttcaaagaagtggcaccattgagatagtgtggggaaggggcccccaa

SEQ ID NO: 38 - DNA, 111 bp, synthetic construct
  misc_feature 1..111: note = 12b-gRNA3-18
  source 1..111: mol_type = other DNA
  modified_base 1..3: mod_base = OTHER; note = 2'-O-methyl nucleotide
  modified_base 1..4: mod_base = OTHER; note = phosphorothioate internucleotide linkage
  modified_base 109..111: mod_base = OTHER; note = 2'-O-methyl nucleotide
  modified_base 108..111: mod_base = OTHER; note = phosphorothioate internucleotide linkage
gcaggtcgtctataggacggcgagtttttcaacgggtgtgccaatggccactttccaggtggcaaagcccgttgagcttcaaagaagtggcacgcattgagatagtgtggg

SEQ ID NO: 39 - DNA, 113 bp, synthetic construct
  misc_feature 1..113: note = 12b-gRNA3-20
  source 1..113: mol_type = other DNA
  modified_base 1..3: mod_base = OTHER; note = 2'-O-methyl nucleotide
  modified_base 1..4: mod_base = OTHER; note = phosphorothioate internucleotide linkage
  modified_base 111..113: mod_base = OTHER; note = 2'-O-methyl nucleotide
  modified_base 110..113: mod_base = OTHER; note = phosphorothioate internucleotide linkage
gcaggtcgtctataggacggcgagtttttcaacgggtgtgccaatggccactttccaggtggcaaagcccgttgagcttcaaagaagtggcacgcattgagatagtgtgggga

SEQ ID NO: 40 - DNA, 114 bp, synthetic construct
  misc_feature 1..114: note = 12b-gRNA3-21
  source 1..114: mol_type = other DNA
  modified_base 1..3: mod_base = OTHER; note = 2'-O-methyl nucleotide
  modified_base 1..4: mod_base = OTHER; note = phosphorothioate internucleotide linkage
  modified_base 112..114: mod_base = OTHER; note = 2'-O-methyl nucleotide
  modified_base 111..114: mod_base = OTHER; note = phosphorothioate internucleotide linkage
gcaggtcgtctataggacggcgagtttttcaacgggtgtgccaatggccactttccaggtggcaaagcccgttgagcttcaaagaagtggcacgcattgagatagtgtggggaa

SEQ ID NO: 41 - DNA, 115 bp, synthetic construct
  misc_feature 1..115: note = 12b-gRNA3-22
  source 1..115: mol_type = other DNA
  modified_base 1..3: mod_base = OTHER; note = 2'-O-methyl nucleotide
  modified_base 1..4: mod_base = OTHER; note = phosphorothioate internucleotide linkage
  modified_base 113..115: mod_base = OTHER; note = 2'-O-methyl nucleotide
  modified_base 112..115: mod_base = OTHER; note = phosphorothioate internucleotide linkage
gcaggtcgtctataggacggcgagtttttcaacgggtgtgccaatggccactttccaggtggcaaagcccgttgagcttcaaagaagtggcacgcattgagatagtgtggggaag

SEQ ID NO: 42 - DNA, 116 bp, synthetic construct
  misc_feature 1..116: note = 12b-gRNA3-23
  source 1..116: mol_type = other DNA
  modified_base 1..3: mod_base = OTHER; note = 2'-O-methyl nucleotide
  modified_base 1..4: mod_base = OTHER; note = phosphorothioate internucleotide linkage
  modified_base 114..116: mod_base = OTHER; note = 2'-O-methyl nucleotide
  modified_base 113..116: mod_base = OTHER; note = phosphorothioate internucleotide linkage
gcaggtcgtctataggacggcgagtttttcaacgggtgtgccaatggccactttccaggtggcaaagcccgttgagcttcaaagaagtggcacgcattgagatagtgtggggaagg

SEQ ID NO: 43 - DNA, 117 bp, synthetic construct
  misc_feature 1..117: note = 12b-gRNA3-24
  source 1..117: mol_type = other DNA
  modified_base 1..3: mod_base = OTHER; note = 2'-O-methyl nucleotide
  modified_base 1..4: mod_base = OTHER; note = phosphorothioate internucleotide linkage
  modified_base 115..117: mod_base = OTHER; note = 2'-O-methyl nucleotide
  modified_base 114..117: mod_base = OTHER; note = phosphorothioate internucleotide linkage
gcaggtcgtctataggacggcgagtttttcaacgggtgtgccaatggccactttccaggtggcaaagcccgttgagcttcaaagaagtggcacgcattgagatagtgtggggaaggg

SEQ ID NO: 44 - DNA, 118 bp, synthetic construct
  misc_feature 1..118: note = 12b-gRNA3-25
  source 1..118: mol_type = other DNA
  modified_base 1..3: mod_base = OTHER; note = 2'-O-methyl nucleotide
  modified_base 1..4: mod_base = OTHER; note = phosphorothioate internucleotide linkage
  modified_base 116..118: mod_base = OTHER; note = 2'-O-methyl nucleotide
  modified_base 115..118: mod_base = OTHER; note = phosphorothioate internucleotide linkage
gcaggtcgtctataggacggcgagtttttcaacgggtgtgccaatggccactttccaggtggcaaagcccgttgagcttcaaagaagtggcacgcattgagatagtgtggggaagggg

SEQ ID NO: 45 - DNA, 119 bp, synthetic construct
  misc_feature 1..119: note = 12b-gRNA3-26
  source 1..119: mol_type = other DNA
  modified_base 1..3: mod_base = OTHER; note = 2'-O-methyl nucleotide
  modified_base 1..4: mod_base = OTHER; note = phosphorothioate internucleotide linkage
  modified_base 117..119: mod_base = OTHER; note = 2'-O-methyl nucleotide
  modified_base 116..119: mod_base = OTHER; note = phosphorothioate internucleotide linkage
gcaggtcgtctataggacggcgagtttttcaacgggtgtgccaatggccactttccaggtggcaaagcccgttgagcttcaaagaagtggcacgcattgagatagtgtggggaaggggc

SEQ ID NO: 46 - DNA, 120 bp, synthetic construct
  misc_feature 1..120: note = 12b-gRNA3-27
  source 1..120: mol_type = other DNA
  modified_base 1..3: mod_base = OTHER; note = 2'-O-methyl nucleotide
  modified_base 1..4: mod_base = OTHER; note = phosphorothioate internucleotide linkage
  modified_base 118..120: mod_base = OTHER; note = 2'-O-methyl nucleotide
  modified_base 117..120: mod_base = OTHER; note = phosphorothioate internucleotide linkage
gcaggtcgtctataggacggcgagtttttcaacgggtgtgccaatggccactttccaggtggcaaagcccgttgagcttcaaagaagtggcacgcattgagatagtgtggggaaggggcc

SEQ ID NO: 47 - DNA, 121 bp, synthetic construct
  misc_feature 1..121: note = 12b-gRNA3-28
  source 1..121: mol_type = other DNA
  modified_base 1..3: mod_base = OTHER; note = 2'-O-methyl nucleotide
  modified_base 1..4: mod_base = OTHER; note = phosphorothioate internucleotide linkage
  modified_base 119..121: mod_base = OTHER; note = 2'-O-methyl nucleotide
  modified_base 118..121: mod_base = OTHER; note = phosphorothioate internucleotide linkage
gcaggtcgtctataggacggcgagtttttcaacgggtgtgccaatggccactttccaggtggcaaagcccgttgagcttcaaagaagtggcacgcattgagatagtgtggggaaggggccc

SEQ ID NO: 48 - DNA, 122 bp, synthetic construct
  misc_feature 1..122: note = 12b-gRNA3-29
  source 1..122: mol_type = other DNA
  modified_base 1..3: mod_base = OTHER; note = 2'-O-methyl nucleotide
  modified_base 1..4: mod_base = OTHER; note = phosphorothioate internucleotide linkage
  modified_base 120..122: mod_base = OTHER; note = 2'-O-methyl nucleotide
  modified_base 119..122: mod_base = OTHER; note = phosphorothioate internucleotide linkage
gcaggtcgtctataggacggcgagtttttcaacgggtgtgccaatggccactttccaggtggcaaagcccgttgagcttcaaagaagtggcacgcattgagatagtgtggggaaggggcccc

SEQ ID NO: 49 - DNA, 123 bp, synthetic construct
  misc_feature 1..123: note = 12b-gRNA3-30
  source 1..123: mol_type = other DNA
  modified_base 1..3: mod_base = OTHER; note = 2'-O-methyl nucleotide
  modified_base 1..4: mod_base = OTHER; note = phosphorothioate internucleotide linkage
  modified_base 121..123: mod_base = OTHER; note = 2'-O-methyl nucleotide
  modified_base 120..123: mod_base = OTHER; note = phosphorothioate internucleotide linkage
gcaggtcgtctataggacggcgagtttttcaacgggtgtgccaatggccactttccaggtggcaaagcccgttgagcttcaaagaagtggcacgcattgagatagtgtggggaaggggccccc

SEQ ID NO: 50 - DNA, 124 bp, synthetic construct
  misc_feature 1..124: note = 12b-gRNA3-31
  source 1..124: mol_type = other DNA
  modified_base 1..3: mod_base = OTHER; note = 2'-O-methyl nucleotide
  modified_base 1..4: mod_base = OTHER; note = phosphorothioate internucleotide linkage
  modified_base 122..124: mod_base = OTHER; note = 2'-O-methyl nucleotide
  modified_base 121..124: mod_base = OTHER; note = phosphorothioate internucleotide linkage
gcaggtcgtctataggacggcgagtttttcaacgggtgtgccaatggccactttccaggtggcaaagcccgttgagcttcaaagaagtggcacgcattgagatagtgtggggaaggggccccca

SEQ ID NO: 51 - DNA, 113 bp, synthetic construct
  misc_feature 1..113: note = 12b-gRNA4
  source 1..113: mol_type = other DNA
  modified_base 1..3: mod_base = OTHER; note = 2'-O-methyl nucleotide
  modified_base 1..4: mod_base = OTHER; note = phosphorothioate internucleotide linkage
  modified_base 111..113: mod_base = OTHER; note = 2'-O-methyl nucleotide
  modified_base 110..113: mod_base = OTHER; note = phosphorothioate internucleotide linkage
gcaggtcgtctataggacggcgagtttttcaacgggtgtgccaatggccactttccaggtggcaaagcccgttgagcttcaaagaagtggcacgccagccttgccttgaccaa

SEQ ID NO: 52 - DNA, 113 bp, synthetic construct
  misc_feature 1..113: note = 12b-gRNA5
  source 1..113: mol_type = other DNA
  modified_base 1..3: mod_base = OTHER; note = 2'-O-methyl nucleotide
  modified_base 1..4: mod_base = OTHER; note = phosphorothioate internucleotide linkage
  modified_base 111..113: mod_base = OTHER; note = 2'-O-methyl nucleotide
  modified_base 110..113: mod_base = OTHER; note = phosphorothioate internucleotide linkage
gcaggtcgtctataggacggcgagtttttcaacgggtgtgccaatggccactttccaggtggcaaagcccgttgagcttcaaagaagtggcacccttgtcaaggctattggtc

SEQ ID NO: 53 - DNA, 113 bp, synthetic construct
  misc_feature 1..113: note = 12b-gRNA6
  source 1..113: mol_type = other DNA
  modified_base 1..3: mod_base = OTHER; note = 2'-O-methyl nucleotide
  modified_base 1..4: mod_base = OTHER; note = phosphorothioate internucleotide linkage
  modified_base 111..113: mod_base = OTHER; note = 2'-O-methyl nucleotide
  modified_base 110..113: mod_base = OTHER; note = phosphorothioate internucleotide linkage
gcaggtcgtctataggacggcgagtttttcaacgggtgtgccaatggccactttccaggtggcaaagcccgttgagcttcaaagaagtggcacgccttgtcaaggctattggt

SEQ ID NO: 54 - DNA, 113 bp, synthetic construct
  misc_feature 1..113: note = 12b-gRNA7
  source 1..113: mol_type = other DNA
  modified_base 1..3: mod_base = OTHER; note = 2'-O-methyl nucleotide
  modified_base 1..4: mod_base = OTHER; note = phosphorothioate internucleotide linkage
  modified_base 111..113: mod_base = OTHER; note = 2'-O-methyl nucleotide
  modified_base 110..113: mod_base = OTHER; note = phosphorothioate internucleotide linkage
gcaggtcgtctataggacggcgagtttttcaacgggtgtgccaatggccactttccaggtggcaaagcccgttgagcttcaaagaagtggcaccagacagatatttgcattga

SEQ ID NO: 55 - DNA, 113 bp, synthetic construct
  misc_feature 1..113: note = 12b-gRNA8
  source 1..113: mol_type = other DNA
  modified_base 1..3: mod_base = OTHER; note = 2'-O-methyl nucleotide
  modified_base 1..4: mod_base = OTHER; note = phosphorothioate internucleotide linkage
  modified_base 111..113: mod_base = OTHER; note = 2'-O-methyl nucleotide
  modified_base 110..113: mod_base = OTHER; note = phosphorothioate internucleotide linkage
gcaggtcgtctataggacggcgagtttttcaacgggtgtgccaatggccactttccaggtggcaaagcccgttgagcttcaaagaagtggcaccccacactatctcaatgcaa

SEQ ID NO: 56 - DNA, 113 bp, synthetic construct
  misc_feature 1..113: note = 12b-gRNA9
  source 1..113: mol_type = other DNA
  modified_base 1..3: mod_base = OTHER; note = 2'-O-methyl nucleotide
  modified_base 1..4: mod_base = OTHER; note = phosphorothioate internucleotide linkage
  modified_base 111..113: mod_base = OTHER; note = 2'-O-methyl nucleotide
  modified_base 110..113: mod_base = OTHER; note = phosphorothioate internucleotide linkage
gcaggtcgtctataggacggcgagtttttcaacgggtgtgccaatggccactttccaggtggcaaagcccgttgagcttcaaagaagtggcacagacagatatttgcattgag

SEQ ID NO: 57 - DNA, 113 bp, synthetic construct
  misc_feature 1..113: note = 12b-gRNA10
  source 1..113: mol_type = other DNA
  modified_base 1..3: mod_base = OTHER; note = 2'-O-methyl nucleotide
  modified_base 1..4: mod_base = OTHER; note = phosphorothioate internucleotide linkage
  modified_base 111..113: mod_base = OTHER; note = 2'-O-methyl nucleotide
  modified_base 110..113: mod_base = OTHER; note = phosphorothioate internucleotide linkage
gcaggtcgtctataggacggcgagtttttcaacgggtgtgccaatggccactttccaggtggcaaagcccgttgagcttcaaagaagtggcactcaaggctattggtcaaggc

SEQ ID NO: 58 - DNA, 113 bp, synthetic construct
  misc_feature 1..113: note = 12b-gRNA11
  source 1..113: mol_type = other DNA
  modified_base 1..3: mod_base = OTHER; note = 2'-O-methyl nucleotide
  modified_base 1..4: mod_base = OTHER; note = phosphorothioate internucleotide linkage
  modified_base 111..113: mod_base = OTHER; note = 2'-O-methyl nucleotide
  modified_base 110..113: mod_base = OTHER; note = phosphorothioate internucleotide linkage
gcaggtcgtctataggacggcgagtttttcaacgggtgtgccaatggccactttccaggtggcaaagcccgttgagcttcaaagaagtggcacagcagcagtatcctcttggg

SEQ ID NO: 59 - DNA, 113 bp, synthetic construct
  misc_feature 1..113: note = 12b-gRNA12
  source 1..113: mol_type = other DNA
  modified_base 1..3: mod_base = OTHER; note = 2'-O-methyl nucleotide
  modified_base 1..4: mod_base = OTHER; note = phosphorothioate internucleotide linkage
  modified_base 111..113: mod_base = OTHER; note = 2'-O-methyl nucleotide
  modified_base 110..113: mod_base = OTHER; note = phosphorothioate internucleotide linkage
gcaggtcgtctataggacggcgagtttttcaacgggtgtgccaatggccactttccaggtggcaaagcccgttgagcttcaaagaagtggcacgtcaagtttgccttgtcaag

SEQ ID NO: 60 - DNA, 107 bp, synthetic construct
  misc_feature 1..107: note = 12b-Aa13tracrRNA
  source 1..107: mol_type = other DNA
  modified_base 1..3: mod_base = OTHER; note = 2'-O-methyl nucleotide
  modified_base 1..4: mod_base = OTHER; note = phosphorothioate internucleotide linkage
  modified_base 105..107: mod_base = OTHER; note = 2'-O-methyl nucleotide
  modified_base 104..107: mod_base = OTHER; note = phosphorothioate internucleotide linkage
ggtcgtctataggacggcgagtttttcaacgggtgtgccaatggccactttccaggtggcaaagcccgttgaacttctcaaaaagaacgctcgctcagtgttctgac

SEQ ID NO: 61 - DNA, 54 bp, synthetic construct
  misc_feature 1..54: note = 12b-crRNA1-18
  source 1..54: mol_type = other DNA
  modified_base 1..3: mod_base = OTHER; note = 2'-O-methyl nucleotide
  modified_base 1..4: mod_base = OTHER; note = phosphorothioate internucleotide linkage
  modified_base 52..54: mod_base = OTHER; note = 2'-O-methyl nucleotide
  modified_base 51..54: mod_base = OTHER; note = phosphorothioate internucleotide linkage
gtcggatcactgagcgagcgatctgagaagtggcacagatagtgtggggaaggg

SEQ ID NO: 62 - DNA, 56 bp, synthetic construct
  misc_feature 1..56: note = 12b-crRNA1-20
  source 1..56: mol_type = other DNA
  modified_base 1..3: mod_base = OTHER; note = 2'-O-methyl nucleotide
  modified_base 1..4: mod_base = OTHER; note = phosphorothioate internucleotide linkage
  modified_base 54..56: mod_base = OTHER; note = 2'-O-methyl nucleotide
  modified_base 53..56: mod_base = OTHER; note = phosphorothioate internucleotide linkage
gtcggatcactgagcgagcgatctgagaagtggcacagatagtgtggggaaggggc

SEQ ID NO: 63 - DNA, 59 bp, synthetic construct
  misc_feature 1..59: note = 12b-crRNA1-23
  source 1..59: mol_type = other DNA
  modified_base 1..3: mod_base = OTHER; note = 2'-O-methyl nucleotide
  modified_base 1..4: mod_base = OTHER; note = phosphorothioate internucleotide linkage
  modified_base 57..59: mod_base = OTHER; note = 2'-O-methyl nucleotide
  modified_base 56..59: mod_base = OTHER; note = phosphorothioate internucleotide linkage
gtcggatcactgagcgagcgatctgagaagtggcacagatagtgtggggaaggggcccc

SEQ ID NO: 64 - DNA, 61 bp, synthetic construct
  misc_feature 1..61: note = 12b-crRNA1-25
  source 1..61: mol_type = other DNA
  modified_base 1..3: mod_base = OTHER; note = 2'-O-methyl nucleotide
  modified_base 1..4: mod_base = OTHER; note = phosphorothioate internucleotide linkage
  modified_base 59..61: mod_base = OTHER; note = 2'-O-methyl nucleotide
  modified_base 58..61: mod_base = OTHER; note = phosphorothioate internucleotide linkage
gtcggatcactgagcgagcgatctgagaagtggcacagatagtgtggggaaggggccccca

SEQ ID NO: 65 - DNA, 64 bp, synthetic construct
  misc_feature 1..64: note = 12b-crRNA1-28
  source 1..64: mol_type = other DNA
  modified_base 1..3: mod_base = OTHER; note = 2'-O-methyl nucleotide
  modified_base 1..4: mod_base = OTHER; note = phosphorothioate internucleotide linkage
  modified_base 62..64: mod_base = OTHER; note = 2'-O-methyl nucleotide
  modified_base 61..64: mod_base = OTHER; note = phosphorothioate internucleotide linkage
gtcggatcactgagcgagcgatctgagaagtggcacagatagtgtggggaaggggcccccaaga

SEQ ID NO: 66 - DNA, 67 bp, synthetic construct
  misc_feature 1..67: note = 12b-crRNA1-31
  source 1..67: mol_type = other DNA
  modified_base 1..3: mod_base = OTHER; note = 2'-O-methyl nucleotide
  modified_base 1..4: mod_base = OTHER; note = phosphorothioate internucleotide linkage
  modified_base 65..67: mod_base = OTHER; note = 2'-O-methyl nucleotide
  modified_base 64..67: mod_base = OTHER; note = phosphorothioate internucleotide linkage
gtcggatcactgagcgagcgatctgagaagtggcacagatagtgtggggaaggggcccccaagagga

SEQ ID NO: 67 - DNA, 43 bp, synthetic construct
  misc_feature 1..43: note = 12i-gRNA-1
  source 1..43: mol_type = other DNA
  modified_base 1..3: mod_base = OTHER; note = 2'-O-methyl nucleotide
  modified_base 1..4: mod_base = OTHER; note = phosphorothioate internucleotide linkage
  modified_base 41..43: mod_base = OTHER; note = 2'-O-methyl nucleotide
  modified_base 40..43: mod_base = OTHER; note = phosphorothioate internucleotide linkage
agaaatccgtctttcattgacggagatagtgtggggaaggggc

SEQ ID NO: 68 - DNA, 43 bp, synthetic construct
  misc_feature 1..43: note = 12i-gRNA-2
  source 1..43: mol_type = other DNA
  modified_base 1..3: mod_base = OTHER; note = 2'-O-methyl nucleotide
  modified_base 1..4: mod_base = OTHER; note = phosphorothioate internucleotide linkage
  modified_base 41..43: mod_base = OTHER; note = 2'-O-methyl nucleotide
  modified_base 40..43: mod_base = OTHER; note = phosphorothioate internucleotide linkage
agaaatccgtctttcattgacggcattgagatagtgtggggaa

SEQ ID NO: 69 - DNA, 43 bp, synthetic construct
  misc_feature 1..43: note = 12i-gRNA-3
  source 1..43: mol_type = other DNA
  modified_base 1..3: mod_base = OTHER; note = 2'-O-methyl nucleotide
  modified_base 1..4: mod_base = OTHER; note = phosphorothioate internucleotide linkage
  modified_base 41..43: mod_base = OTHER; note = 2'-O-methyl nucleotide
  modified_base 40..43: mod_base = OTHER; note = phosphorothioate internucleotide linkage
agaaatccgtctttcattgacgggcattgagatagtgtgggga

SEQ ID NO: 70 - DNA, 43 bp, synthetic construct
  misc_feature 1..43: note = 12i-gRNA-4
  source 1..43: mol_type = other DNA
  modified_base 1..3: mod_base = OTHER; note = 2'-O-methyl nucleotide
  modified_base 1..4: mod_base = OTHER; note = phosphorothioate internucleotide linkage
  modified_base 41..43: mod_base = OTHER; note = 2'-O-methyl nucleotide
  modified_base 40..43: mod_base = OTHER; note = phosphorothioate internucleotide linkage
agaaatccgtctttcattgacgggccagccttgccttgaccaa

SEQ ID NO: 71 - DNA, 43 bp, synthetic construct
  misc_feature 1..43: note = 12i-gRNA-5
  source 1..43: mol_type = other DNA
  modified_base 1..3: mod_base = OTHER; note = 2'-O-methyl nucleotide
  modified_base 1..4: mod_base = OTHER; note = phosphorothioate internucleotide linkage
  modified_base 41..43: mod_base = OTHER; note = 2'-O-methyl nucleotide
  modified_base 40..43: mod_base = OTHER; note = phosphorothioate internucleotide linkage
agaaatccgtctttcattgacggccttgtcaaggctattggtc

SEQ ID NO: 72 - DNA, 43 bp, synthetic construct
  misc_feature 1..43: note = 12i-gRNA-6
  source 1..43: mol_type = other DNA
  modified_base 1..3: mod_base = OTHER; note = 2'-O-methyl nucleotide
  modified_base 1..4: mod_base = OTHER; note = phosphorothioate internucleotide linkage
  modified_base 41..43: mod_base = OTHER; note = 2'-O-methyl nucleotide
  modified_base 40..43: mod_base = OTHER; note = phosphorothioate internucleotide linkage
agaaatccgtctttcattgacgggccttgtcaaggctattggt

SEQ ID NO: 73 - DNA, 43 bp, synthetic construct
  misc_feature 1..43: note = 12i-gRNA-7
  source 1..43: mol_type = other DNA
  modified_base 1..3: mod_base = OTHER; note = 2'-O-methyl nucleotide
  modified_base 1..4: mod_base = OTHER; note = phosphorothioate internucleotide linkage
  modified_base 41..43: mod_base = OTHER; note = 2'-O-methyl nucleotide
  modified_base 40..43: mod_base = OTHER; note = phosphorothioate internucleotide linkage
agaaatccgtctttcattgacggcagacagatatttgcattga

SEQ ID NO: 74 - DNA, 43 bp, synthetic construct
  misc_feature 1..43: note = 12i-gRNA-8
  source 1..43: mol_type = other DNA
  modified_base 1..3: mod_base = OTHER; note = 2'-O-methyl nucleotide
  modified_base 1..4: mod_base = OTHER; note = phosphorothioate internucleotide linkage
  modified_base 41..43: mod_base = OTHER; note = 2'-O-methyl nucleotide
  modified_base 40..43: mod_base = OTHER; note = phosphorothioate internucleotide linkage
agaaatccgtctttcattgacggcccacactatctcaatgcaa

SEQ ID NO: 75 - DNA, 43 bp, synthetic construct
  misc_feature 1..43: note = 12i-gRNA-9
  source 1..43: mol_type = other DNA
  modified_base 1..3: mod_base = OTHER; note = 2'-O-methyl nucleotide
  modified_base 1..4: mod_base = OTHER; note = phosphorothioate internucleotide linkage
  modified_base 41..43: mod_base = OTHER; note = 2'-O-methyl nucleotide
  modified_base 40..43: mod_base = OTHER; note = phosphorothioate internucleotide linkage
agaaatccgtctttcattgacggagacagatatttgcattgag

SEQ ID NO: 76 - DNA, 43 bp, synthetic construct
  misc_feature 1..43: note = 12i-gRNA-10
  source 1..43: mol_type = other DNA
  modified_base 1..3: mod_base = OTHER; note = 2'-O-methyl nucleotide
  modified_base 1..4: mod_base = OTHER; note = phosphorothioate internucleotide linkage
  modified_base 41..43: mod_base = OTHER; note = 2'-O-methyl nucleotide
  modified_base 40..43: mod_base = OTHER; note = phosphorothioate internucleotide linkage
agaaatccgtctttcattgacggtcaaggctattggtcaaggc

SEQ ID NO: 77 - DNA, 43 bp, synthetic construct
  misc_feature 1..43: note = 12i-gRNA-11
  source 1..43: mol_type = other DNA
  modified_base 1..3: mod_base = OTHER; note = 2'-O-methyl nucleotide
  modified_base 1..4: mod_base = OTHER; note = phosphorothioate internucleotide linkage
  modified_base 41..43: mod_base = OTHER; note = 2'-O-methyl nucleotide
  modified_base 40..43: mod_base = OTHER; note = phosphorothioate internucleotide linkage
agaaatccgtctttcattgacggagcagcagtatcctcttggg

SEQ ID NO: 78 - DNA, 43 bp, synthetic construct
  misc_feature 1..43: note = 12i-gRNA-12
  source 1..43: mol_type = other DNA
  modified_base 1..3: mod_base = OTHER; note = 2'-O-methyl nucleotide
  modified_base 1..4: mod_base = OTHER; note = phosphorothioate internucleotide linkage
  modified_base 41..43: mod_base = OTHER; note = 2'-O-methyl nucleotide
  modified_base 40..43: mod_base = OTHER; note = phosphorothioate internucleotide linkage
agaaatccgtctttcattgacgggtcaagtttgccttgtcaag

SEQ ID NO: 79 - DNA, 3465 bp, synthetic construct
  misc_feature 1..3465: note = Ecoli Cas12b-M1
  source 1..3465: mol_type = other DNA
atgcatcatcatcatcaccatccgaaaaagaaacgcaaagttccgggcatggcagtgaaaagtatgaaagtgaaactgcgtctggataatatgccggaaattcgtgcaggcctgtggaaactgcataccgaagttaatgccggcgttcgctattataccgaatggctgagtctgctgcgtcaggaaaatctgtatcgtcgcagtccgaatggcgatggtgaacaggaatgctataaaaccgccgaagaatgcaaagccgaactgctggaacgtctgcgcgcccgccaggttgaaaatggtcattgcggtccggcaggtagcgatgatgaactgctgcagctggcacgccagctgtatgaactgctggttccgcaggcaattggtgccaaaggtgacgcccagtttattgcccgcaaatttctgagtccgctggccgataaagatgccgtgggtggcctgggtattgccaaagccggcaataagccgcgttgggttcgcatgcgtgaagccggcgaaccgggttgggaagaagaaaaagcaaaagccgaagcacgtaaaagcaccgatcgcaccgcagatgttctgcgtgcactggcagattttggtctgaaaccgctgatgcgtgtttataccgatagcgatatgagcagcgtgcagtggaaaccgctgcgcaaaggccaggccgtgcgcacatgggatcgtgatatgtttcagcaggccattgaacgtatgatgagttgggaaagttggaatcagcgtgtgggtgaagcctatgcaaaactggtggaacagaaaagtcgttttgaacagaaaaatttcgtgggtcaggaacatctggttcagctggtgaatcagctgcagcaggatatgaaagaagcaagccacggtctggaaagcaaagaacagaccgcacattatctgaccggccgtgccctgcgcggcagtgataaagtgtttgaaaaatgggaaaagctggaccctgatgcaccgtttgatctgtatgataccgaaattaagaacgtgcagcgccgtaatacccgccgctttggtagtcatgatctgtttgccaaactggcagaaccgaaatatcaggcactgtggcgcgaagatgccagttttctgacccgttatgccgtttataatagcattgtgcgcaaactgaatcatgccaaaatgtttgccacctttaccctgccggatgcaaccgcacatccgatttggacccgctttgataaactgggtggtaatctgcatcagtatacctttctgtttaatgaatttggtgagggccgtcatgcaattcgctttcagaaactgctgaccgtggaagatggcgtggcaaaagaagtggatgatgtgaccgtgccgattagcatgagcgcacagctggatgatctgctgccgcgtgatccgcatgaactggtggcactgtattttcaggattatggtgcagaacagcatctggccggccgttttggtggtgccaaaattcagtatcgccgtgatcagctgaatcatctgcatgcccgccgtggcgcccgtgatgtttatctgaatctgagcgttcgcgttcagagtcagagcgaagcacgtggtgaacgccgtccgccgtatgcagccgtgtttcgcctggttggcgataatcatcgcgcatttgtgcattttgataaattaagtgactacctggcagaacatccggatgatggtaaactgggtagtgaaggcctgctgagtggcctgcgtgttatgagtgtggatctgggcctgcgtaccagcgcaagtattagtgtgtttcgtgtggcacgtaaagatgaactgaaaccgaatagtgaaggccgcgttccgttttgttttccgattgaaggcaatgaaaatctggttgcagttcatgaacgcagccagctgctgaaactgccgggcgaaaccgaaagcaaagatctgcgcgcaattcgcgaagaacgtcagcgcaccctgcgtcagctgcgtacccagctggcctatctgcgcctgctggtgcgttgtggcagcgaagatgttggccgtcgtgaacgcagctgggcaaaactgattgaacagccgatggatgcaaatcagatgaccccggattggcgcgaagcatttgaagatgaactgcagaaactgaaaagtctgtatggcatttgtggtgaccgtgaatggaccgaagccgtgtatgaaagcgttcgccgcgtttggcgccacatgggcaaacaggttcgcgattggcgcaaagatgttcgtagcggcgaacgtccgaaaattcgtggttatcagaaagatgtggttggcggcaatagcattcgccagattgaatatctggaacgtcagtataaattcctgaaaagttggagctttttcggtaaagtgagtggtcaggttattcgtgccgaaaaaggtagtcgctttgcaattaccctgcgcgaacatattgatcatgccaaagaagatcgtctgaaaaaactggcagatcgtattattatggaagccctgggttatgtgtatgccctggatgatgaacgtggtaaaggcaaatgggtggcaaaatatccgccgtgccagctgattctgctggaagaactgagcgaatatcagtttaataatgatcgcccgccgagtgaaaataatcagctgatgcagtggagccatcgtggtgtgtttcaggaactgctgaatcaggcacaggttcatgatctgctggttggcaccatgtatgcagcctttagtagccgttttgatgcacgtaccggcgcaccgggtattcgttgtcgtcgcgttccggcccgctgcgctcgtgaacagaatccggaaccgtttccgtggtggctgaataagtttgtggccgaacataaactggatggttgtccgctgcgcgcagatgatctgattccgaccggtgaaggtgaatttttcgttagcccgtttagtgccgaagaaggtgactttcatcagattcatgccgatctgaatgccgcacagaatctgcagcgccgtctgtggagcgattttgatattagtcagattcgtctgcgttgtgattggggtgaagtggatggtgaaccggtgctgattccgcgtaccaccggtaaacgcaccgccgatagttatggcaataaggtgttttataccaaaaccggcgttacctattatgaacgtgaacgcggcaaaaaacgtcgcaaagtttttgcccaggaagaactgagtgaagaagaagccgaactgttagtggaagcagatgaagcacgtgaaaaaagcgtggtgctgatgcgcgatccgagtggtattattaatcgcggtgactggacccgtcagaaagaattttggagcatggttaatcagcgcattgaaggttatctggtgaaacagattcgtagccgtgttcgtctgcaggaaagtgcctgtgaaaataccggtgacattgcaagtccgaaaaagaaacgtaaagtttaa

SEQ ID NO: 80 - DNA, 3447 bp, synthetic construct
  misc_feature 1..3447: note = Ecoli Cas12b-M2
  source 1..3447: mol_type = other DNA
atgccgaaaaagaaacgcaaagttccgggcatggcagtgaaaagtatgaaagtgaaactgcgtctggataatatgccggaaattcgtgcaggcctgtggaaactgcataccgaagttaatgccggcgttcgctattataccgaatggctgagtctgctgcgtcaggaaaatctgtatcgtcgcagtccgaatggcgatggtgaacaggaatgctataaaaccgccgaagaatgcaaagccgaactgctggaacgtctgcgcgcccgccaggttgaaaatggtcattgcggtccggcaggtagcgatgatgaactgctgcagctggcacgccagctgtatgaactgctggttccgcaggcaattggtgccaaaggtgacgcccagtttattgcccgcaaatttctgagtccgctggccgataaagatgccgtgggtggcctgggtattgccaaagccggcaataagccgcgttgggttcgcatgcgtgaagccggcgaaccgggttgggaagaagaaaaagcaaaagccgaagcacgtaaaagcaccgatcgcaccgcagatgttctgcgtgcactggcagattttggtctgaaaccgctgatgcgtgtttataccgatagcgatatgagcagcgtgcagtggaaaccgctgcgcaaaggccaggccgtgcgcacatgggatcgtgatatgtttcagcaggccattgaacgtatgatgagttgggaaagttggaatcagcgtgtgggtgaagcctatgcaaaactggtggaacagaaaagtcgttttgaacagaaaaatttcgtgggtcaggaacatctggttcagctggtgaatcagctgcagcaggatatgaaagaagcaagccacggtctggaaagcaaagaacagaccgcacattatctgaccggccgtgccctgcgcggcagtgataaagtgtttgaaaaatgggaaaagctggaccctgatgcaccgtttgatctgtatgataccgaaattaagaacgtgcagcgccgtaatacccgccgctttggtagtcatgatctgtttgccaaactggcagaaccgaaatatcaggcactgtggcgcgaagatgccagttttctgacccgttatgccgtttataatagcattgtgcgcaaactgaatcatgccaaaatgtttgccacctttaccctgccggatgcaaccgcacatccgatttggacccgctttgataaactgggtggtaatctgcatcagtatacctttctgtttaatgaatttggtgagggccgtcatgcaattcgctttcagaaactgctgaccgtggaagatggcgtggcaaaagaagtggatgatgtgaccgtgccgattagcatgagcgcacagctggatgatctgctgccgcgtgatccgcatgaactggtggcactgtattttcaggattatggtgcagaacagcatctggccggccgttttggtggtgccaaaattcagtatcgccgtgatcagctgaatcatctgcatgcccgccgtggcgcccgtgatgtttatctgaatctgagcgttcgcgttcagagtcagagcgaagcacgtggtgaacgccgtccgccgtatgcagccgtgtttcgcctggttggcgataatcatcgcgcatttgtgcattttgataaattaagtgactacctggcagaacatccggatgatggtaaactgggtagtgaaggcctgctgagtggcctgcgtgttatgagtgtggatctgggcctgcgtaccagcgcaagtattagtgtgtttcgtgtggcacgtaaagatgaactgaaaccgaatagtgaaggccgcgttccgttttgttttccgattgaaggcaatgaaaatctggttgcagttcatgaacgcagccagctgctgaaactgccgggcgaaaccgaaagcaaagatctgcgcgcaattcgcgaagaacgtcagcgcaccctgcgtcagctgcgtacccagctggcctatctgcgcctgctggtgcgttgtggcagcgaagatgttggccgtcgtgaacgcagctgggcaaaactgattgaacagccgatggatgcaaatcagatgaccccggattggcgcgaagcatttgaagatgaactgcagaaactgaaaagtctgtatggcatttgtggtgaccgtgaatggaccgaagccgtgtatgaaagcgttcgccgcgtttggcgccacatgggcaaacaggttcgcgattggcgcaaagatgttcgtagcggcgaacgtccgaaaattcgtggttatcagaaagatgtggttggcggcaatagcattcgccagattgaatatctggaacgtcagtataaattcctgaaaagttggagctttttcggtaaagtgagtggtcaggttattcgtgccgaaaaaggtagtcgctttgcaattaccctgcgcgaacatattgatcatgccaaagaagatcgtctgaaaaaactggcagatcgtattattatggaagccctgggttatgtgtatgccctggatgatgaacgtggtaaaggcaaatgggtggcaaaatatccgccgtgccagctgattctgctggaagaactgagcgaatatcagtttaataatgatcgcccgccgagtgaaaataatcagctgatgcagtggagccatcgtggtgtgtttcaggaactgctgaatcaggcacaggttcatgatctgctggttggcaccatgtatgcagcctttagtagccgttttgatgcacgtaccggcgcaccgggtattcgttgtcgtcgcgttccggcccgctgcgctcgtgaacagaatccggaaccgtttccgtggtggctgaataagtttgtggccgaacataaactggatggttgtccgctgcgcgcagatgatctgattccgaccggtgaaggtgaatttttcgttagcccgtttagtgccgaagaaggtgactttcatcagattcatgccgatctgaatgccgcacagaatctgcagcgccgtctgtggagcgattttgatattagtcagattcgtctgcgttgtgattggggtgaagtggatggtgaaccggtgctgattccgcgtaccaccggtaaacgcaccgccgatagttatggcaataaggtgttttataccaaaaccggcgttacctattatgaacgtgaacgcggcaaaaaacgtcgcaaagtttttgcccaggaagaactgagtgaagaagaagccgaactgttagtggaagcagatgaagcacgtgaaaaaagcgtggtgctgatgcgcgatccgagtggtattattaatcgcggtgactggacccgtcagaaagaattttggagcatggttaatcagcgcattgaaggttatctggtgaaacagattcgtagccgtgttcgtctgcaggaaagtgcctgtgaaaataccggtgacattgcaagtccgaaaaagaaacgtaaagtttaa

SEQ ID NO: 81 - DNA, 3495 bp, synthetic construct
  misc_feature 1..3495: note = Ecoli Cas12b-M3
  source 1..3495: mol_type = other DNA
atgccgaaaaaaaagcgtaaagttccgggcatggcagtgaaaagtatgaaagtgaaactgcgtctggataatatgccggaaattcgtgcaggcctgtggaaactgcataccgaagttaatgccggcgttcgctattataccgaatggctgagtctgctgcgtcaggaaaatctgtatcgtcgcagtccgaatggcgatggtgaacaggaatgctataaaaccgccgaagaatgcaaagccgaactgctggaacgtctgcgcgcccgccaggttgaaaatggtcattgcggtccggcaggtagcgatgatgaactgctgcagctggcacgccagctgtatgaactgctggttccgcaggcaattggtgccaaaggtgacgcccagtttattgcccgcaaatttctgagtccgctggccgataaagatgccgtgggtggcctgggtattgccaaagccggcaataagccgcgttgggttcgcatgcgtgaagccggcgaaccgggttgggaagaagaaaaagcaaaagccgaagcacgtaaaagcaccgatcgcaccgcagatgttctgcgtgcactggcagattttggtctgaaaccgctgatgcgtgtttataccgatagcgatatgagcagcgtgcagtggaaaccgctgcgcaaaggccaggccgtgcgcacatgggatcgtgatatgtttcagcaggccattgaacgtatgatgagttgggaaagttggaatcagcgtgtgggtgaagcctatgcaaaactggtggaacagaaaagtcgttttgaacagaaaaatttcgtgggtcaggaacatctggttcagctggtgaatcagctgcagcaggatatgaaagaagcaagccacggtctggaaagcaaagaacagaccgcacattatctgaccggccgtgccctgcgcggcagtgataaagtgtttgaaaaatgggaaaagctggaccctgatgcaccgtttgatctgtatgataccgaaattaagaacgtgcagcgccgtaatacccgccgctttggtagtcatgatctgtttgccaaactggcagaaccgaaatatcaggcactgtggcgcgaagatgccagttttctgacccgttatgccgtttataatagcattgtgcgcaaactgaatcatgccaaaatgtttgccacctttaccctgccggatgcaaccgcacatccgatttggacccgctttgataaactgggtggtaatctgcatcagtatacctttctgtttaatgaatttggtgagggccgtcatgcaattcgctttcagaaactgctgaccgtggaagatggcgtggcaaaagaagtggatgatgtgaccgtgccgattagcatgagcgcacagctggatgatctgctgccgcgtgatccgcatgaactggtggcactgtattttcaggattatggtgcagaacagcatctggccggccgttttggtggtgccaaaattcagtatcgccgtgatcagctgaatcatctgcatgcccgccgtggcgcccgtgatgtttatctgaatctgagcgttcgcgttcagagtcagagcgaagcacgtggtgaacgccgtccgccgtatgcagccgtgtttcgcctggttggcgataatcatcgcgcatttgtgcattttgataaattaagtgactacctggcagaacatccggatgatggtaaactgggtagtgaaggcctgctgagtggcctgcgtgttatgagtgtggatctgggcctgcgtaccagcgcaagtattagtgtgtttcgtgtggcacgtaaagatgaactgaaaccgaatagtgaaggccgcgttccgttttgttttccgattgaaggcaatgaaaatctggttgcagttcatgaacgcagccagctgctgaaactgccgggcgaaaccgaaagcaaagatctgcgcgcaattcgcgaagaacgtcagcgcaccctgcgtcagctgcgtacccagctggcctatctgcgcctgctggtgcgttgtggcagcgaagatgttggccgtcgtgaacgcagctgggcaaaactgattgaacagccgatggatgcaaatcagatgaccccggattggcgcgaagcatttgaagatgaactgcagaaactgaaaagtctgtatggcatttgtggtgaccgtgaatggaccgaagccgtgtatgaaagcgttcgccgcgtttggcgccacatgggcaaacaggttcgcgattggcgcaaagatgttcgtagcggcgaacgtccgaaaattcgtggttatcagaaagatgtggttggcggcaatagcattcgccagattgaatatctggaacgtcagtataaattcctgaaaagttggagctttttcggtaaagtgagtggtcaggttattcgtgccgaaaaaggtagtcgctttgcaattaccctgcgcgaacatattgatcatgccaaagaagatcgtctgaaaaaactggcagatcgtattattatggaagccctgggttatgtgtatgccctggatgatgaacgtggtaaaggcaaatgggtggcaaaatatccgccgtgccagctgattctgctggaagaactgagcgaatatcagtttaataatgatcgcccgccgagtgaaaataatcagctgatgcagtggagccatcgtggtgtgtttcaggaactgctgaatcaggcacaggttcatgatctgctggttggcaccatgtatgcagcctttagtagccgttttgatgcacgtaccggcgcaccgggtattcgttgtcgtcgcgttccggcccgctgcgctcgtgaacagaatccggaaccgtttccgtggtggctgaataagtttgtggccgaacataaactggatggttgtccgctgcgcgcagatgatctgattccgaccggtgaaggtgaatttttcgttagcccgtttagtgccgaagaaggtgactttcatcagattcatgccgatctgaatgccgcacagaatctgcagcgccgtctgtggagcgattttgatattagtcagattcgtctgcgttgtgattggggtgaagtggatggtgaaccggtgctgattccgcgtaccaccggtaaacgcaccgccgatagttatggcaataaggtgttttataccaaaaccggcgttacctattatgaacgtgaacgcggcaaaaaacgtcgcaaagtttttgcccaggaagaactgagtgaagaagaagccgaactgttagtggaagcagatgaagcacgtgaaaaaagcgtggtgctgatgcgcgatccgagtggtattattaatcgcggtgactggacccgtcagaaagaattttggagcatggttaatcagcgcattgaaggttatctggtgaaacagattcgtagccgtgttcgtctgcaggaaagtgcctgtgaaaataccggtgacattgcaagtcctaaaaagaagcgtaaagtcaaacgtccagcagcaaccaaaaaagcaggccaagcaaaaaaaaaaaagtaa

SEQ ID NO: 82 - DNA, 3474 bp, synthetic construct
  misc_feature 1..3474: note = Ecoli Cas12b-M4
  source 1..3474: mol_type = other DNA
atgccgaaaaaaaagcgtaaagttccgggcatggcagtgaaaagtatgaaagtgaaactgcgtctggataatatgccggaaattcgtgcaggcctgtggaaactgcataccgaagttaatgccggcgttcgctattataccgaatggctgagtctgctgcgtcaggaaaatctgtatcgtcgcagtccgaatggcgatggtgaacaggaatgctataaaaccgccgaagaatgcaaagccgaactgctggaacgtctgcgcgcccgccaggttgaaaatggtcattgcggtccggcaggtagcgatgatgaactgctgcagctggcacgccagctgtatgaactgctggttccgcaggcaattggtgccaaaggtgacgcccagtttattgcccgcaaatttctgagtccgctggccgataaagatgccgtgggtggcctgggtattgccaaagccggcaataagccgcgttgggttcgcatgcgtgaagccggcgaaccgggttgggaagaagaaaaagcaaaagccgaagcacgtaaaagcaccgatcgcaccgcagatgttctgcgtgcactggcagattttggtctgaaaccgctgatgcgtgtttataccgatagcgatatgagcagcgtgcagtggaaaccgctgcgcaaaggccaggccgtgcgcacatgggatcgtgatatgtttcagcaggccattgaacgtatgatgagttgggaaagttggaatcagcgtgtgggtgaagcctatgcaaaactggtggaacagaaaagtcgttttgaacagaaaaatttcgtgggtcaggaacatctggttcagctggtgaatcagctgcagcaggatatgaaagaagcaagccacggtctggaaagcaaagaacagaccgcacattatctgaccggccgtgccctgcgcggcagtgataaagtgtttgaaaaatgggaaaagctggaccctgatgcaccgtttgatctgtatgataccgaaattaagaacgtgcagcgccgtaatacccgccgctttggtagtcatgatctgtttgccaaactggcagaaccgaaatatcaggcactgtggcgcgaagatgccagttttctgacccgttatgccgtttataatagcattgtgcgcaaactgaatcatgccaaaatgtttgccacctttaccctgccggatgcaaccgcacatccgatttggacccgctttgataaactgggtggtaatctgcatcagtatacctttctgtttaatgaatttggtgagggccgtcatgcaattcgctttcagaaactgctgaccgtggaagatggcgtggcaaaagaagtggatgatgtgaccgtgccgattagcatgagcgcacagctggatgatctgctgccgcgtgatccgcatgaactggtggcactgtattttcaggattatggtgcagaacagcatctggccggccgttttggtggtgccaaaattcagtatcgccgtgatcagctgaatcatctgcatgcccgccgtggcgcccgtgatgtttatctgaatctgagcgttcgcgttcagagtcagagcgaagcacgtggtgaacgccgtccgccgtatgcagccgtgtttcgcctggttggcgataatcatcgcgcatttgtgcattttgataaattaagtgactacctggcagaacatccggatgatggtaaactgggtagtgaaggcctgctgagtggcctgcgtgttatgagtgtggatctgggcctgcgtaccagcgcaagtattagtgtgtttcgtgtggcacgtaaagatgaactgaaaccgaatagtgaaggccgcgttccgttttgttttccgattgaaggcaatgaaaatctggttgcagttcatgaacgcagccagctgctgaaactgccgggcgaaaccgaaagcaaagatctgcgcgcaattcgcgaagaacgtcagcgcaccctgcgtcagctgcgtacccagctggcctatctgcgcctgctggtgcgttgtggcagcgaagatgttggccgtcgtgaacgcagctgggcaaaactgattgaacagccgatggatgcaaatcagatgaccccggattggcgcgaagcatttgaagatgaactgcagaaactgaaaagtctgtatggcatttgtggtgaccgtgaatggaccgaagccgtgtatgaaagcgttcgccgcgtttggcgccacatgggcaaacaggttcgcgattggcgcaaagatgttcgtagcggcgaacgtccgaaaattcgtggttatcagaaagatgtggttggcggcaatagcattcgccagattgaatatctggaacgtcagtataaattcctgaaaagttggagctttttcggtaaagtgagtggtcaggttattcgtgccgaaaaaggtagtcgctttgcaattaccctgcgcgaacatattgatcatgccaaagaagatcgtctgaaaaaactggcagatcgtattattatggaagccctgggttatgtgtatgccctggatgatgaacgtggtaaaggcaaatgggtggcaaaatatccgccgtgccagctgattctgctggaagaactgagcgaatatcagtttaataatgatcgcccgccgagtgaaaataatcagctgatgcagtggagccatcgtggtgtgtttcaggaactgctgaatcaggcacaggttcatgatctgctggttggcaccatgtatgcagcctttagtagccgttttgatgcacgtaccggcgcaccgggtattcgttgtcgtcgcgttccggcccgctgcgctcgtgaacagaatccggaaccgtttccgtggtggctgaataagtttgtggccgaacataaactggatggttgtccgctgcgcgcagatgatctgattccgaccggtgaaggtgaatttttcgttagcccgtttagtgccgaagaaggtgactttcatcagattcatgccgatctgaatgccgcacagaatctgcagcgccgtctgtggagcgattttgatattagtcagattcgtctgcgttgtgattggggtgaagtggatggtgaaccggtgctgattccgcgtaccaccggtaaacgcaccgccgatagttatggcaataaggtgttttataccaaaaccggcgttacctattatgaacgtgaacgcggcaaaaaacgtcgcaaagtttttgcccaggaagaactgagtgaagaagaagccgaactgttagtggaagcagatgaagcacgtgaaaaaagcgtggtgctgatgcgcgatccgagtggtattattaatcgcggtgactggacccgtcagaaagaattttggagcatggttaatcagcgcattgaaggttatctggtgaaacagattcgtagccgtgttcgtctgcaggaaagtgcctgtgaaaataccggtgacattgcaagtcctaaaaagaagcgtaaagtcccagcagcaaaaaaaaaaaagttagattaa

SEQ ID NO: 83 - DNA, 3546 bp, synthetic construct
  misc_feature 1..3546: note = Ecoli Cas12b-M5
  source 1..3546: mol_type = other DNA
atgcctgcagccaaaaagaaaaagctggatggtagcggtagcccgaaaaagaaacgtaaagttcctggtatggcagtcaaaagcatgaaagttaaactgcgcctggataacatgccggaaattcgtgcaggtctgtggaaactgcataccgaagttaatgccggtgttcgttattataccgaatggctgagcctgctgcgtcaagaaaatctgtatcgtcgtagtccgaatggtgatggtgaacaagaatgttataaaaccgcagaagaatgcaaagcagaactgctggaacgtctgcgtgcacgtcaggttgaaaatggtcattgtggtccggcaggtagtgatgatgaactgctgcagctggcacgtcagctgtatgagctgctggttccgcaggcaattggtgcaaaaggtgatgcacagtttattgcccgtaaatttctgagtccgctggcagataaagatgcagttggtggtctgggtattgcaaaagcaggtaataaaccgcgttgggttcgtatgcgtgaagccggtgaacctggttgggaagaagagaaagccaaagccgaagcacgtaaaagcaccgatcgtaccgcagatgttctgcgtgccctggcagattttggtctgaaaccgctgatgcgtgtttataccgatagcgatatgagcagcgttcagtggaaacctctgcgtaaaggtcaggcagttcgtacctgggatcgtgatatgtttcagcaggccattgaacgtatgatgagctgggaaagctggaatcagcgtgttggtgaagcctatgcaaaactggttgaacagaaaagccgtttcgagcagaaaaactttgttggtcaagaacacctggttcagctggtgaatcagctgcaacaggatatgaaagaagcaagccacggtctggaaagcaaagaacagaccgcacattatctgaccggtcgtgcactgcgtggtagcgataaagtttttgaaaaatgggaaaaactggatccggatgcaccgtttgatctgtatgataccgaaatcaaaaatgtgcagcgtcgtaatacccgtcgttttggtagccatgacctgtttgccaaactggcagaaccgaaatatcaggcactgtggcgtgaagatgcaagctttctgacccgttatgcagtgtataatagcattgtgcgcaaactgaatcacgccaaaatgtttgcaacctttacactgccggatgcaaccgcacatccgatttggacccgttttgataaattaggtggtaacctgcaccagtacacctttctgtttaatgaatttggtgaaggtcgtcatgccatccgttttcagaaactgctgaccgttgaagatggtgttgcaaaagaagttgacgacgttaccgttccgattagcatgagcgcacagctggatgatctgcttccgcgtgatccgcatgaactggttgcactgtattttcaggattatggtgcagaacagcatctggcaggtcgctttggtggtgccaaaattcagtatcgtcgcgatcagctgaatcatctgcatgcccgtcgtggtgcacgtgatgtttatctgaatctgagcgttcgtgttcagagccagagcgaagcccgtggtgaacgtcgccctccgtatgcagccgtttttcgtctggttggtgataatcatcgtgcctttgttcactttgataaactgagcgattatctggccgaacatcctgatgatggtaaactgggtagcgaaggtctgctgagcggtctgcgtgttatgagcgttgatctgggtctgcgtaccagcgcaagcattagcgtgtttcgtgttgcacgtaaagatgaactgaaaccgaatagcgaaggccgtgttccgttttgttttccgattgaaggtaatgaaaatctggttgcagtgcatgaacgtagtcagctgctgaaattaccgggtgaaacagaatcaaaagatctgcgtgcgattcgtgaagaacgtcagcgtaccctgcgtcagctgcgcacccagctggcatatctgcgtctgctggtgcgttgtggtagtgaagatgttggtcgtcgtgaacgtagctgggccaaactgatcgaacagccgatggatgcaaatcagatgacaccggattggcgtgaggcatttgaagatgagctgcagaaactgaaaagcctgtatggtatttgtggtgatcgtgaatggaccgaagccgtttatgaaagcgttcgtcgtgtttggcgtcacatgggtaaacaggttcgtgattggcgcaaagatgttcgtagtggcgaacgtccgaaaattcgtggttatcagaaagatgttgttggtggcaatagcattcgccagattgaatatctggaacgccagtacaaattcctgaaaagctggtcatttttcggtaaagttagcggtcaggttattcgtgccgaaaaaggtagccgttttgcaattacactgcgcgaacatattgatcatgccaaagaagatcgtctgaagaaactggccgatcgcattattatggaagcactgggttatgtttatgccctggatgatgaacgtggtaaaggtaaatgggttgccaaatatccgccttgccagctgatcctgctggaagaactgagtgaatatcagtttaataacgatcgtccgcctagcgaaaataaccagctgatgcagtggtcccatcgtggtgtttttcaagaactgttaaatcaggcacaggttcacgatctgctggttggcaccatgtatgcagcatttagcagtcgttttgatgcacgtacaggtgcaccgggtattcgttgccgtcgtgttccggcacgttgtgcccgtgaacagaatccggaaccgtttccgtggtggctgaataaattcgttgcagaacataaactggatggttgtccgctgcgtgccgatgatctgatcccgaccggtgaaggtgaatttttcgttagcccgttttctgccgaagaaggtgattttcatcagattcatgcagatctgaatgcagcacagaatctgcaacgtcgtctgtggtcagattttgatatcagccagattcgtctgcgctgtgattggggtgaagttgatggcgaaccggtgctgattccgcgtaccaccggtaaacgtacagcagatagctatggtaacaaagtgttctataccaaaaccggtgtgacctattatgaacgtgaacgcggtaagaaacgtcgtaaagtgtttgcacaagaagaactgtcagaagaagaagccgaactgttagttgaagcagatgaagcgcgtgaaaaatcagttgttctgatgcgcgatccgagcggtattatcaatcgtggtgattggacacgtcagaaagaattttggagcatggttaatcagcgcattgaaggttatctggtgaaacaaattcgtagccgtgttcgtctgcaagaatcagcatgtgaaaataccggtgatattgcaagccctaagaagaaaagaaaagttggtagtggtagcaaacgtccggcagcaaccaaaaaggcaggtcaggctaaaaagaagaaataa

SEQ ID NO: 84 - DNA, 3525 bp, synthetic construct
  misc_feature 1..3525: note = Ecoli Cas12b-M6
  source 1..3525: mol_type = other DNA
atgcctggtatggcagtgaaaagcatgaaagttaaactgcgcctggataacatgccggaaattcgtgcaggtctgtggaaactgcataccgaagttaatgccggtgttcgttattataccgaatggctgagcctgctgcgtcaagaaaatctgtatcgtcgtagcccgaatggtgatggtgaacaagaatgttataaaaccgcagaagaatgcaaagcagaactgctggaacgtctgcgtgcacgtcaggttgaaaatggtcattgtggtccggcaggtagtgatgatgaactgctgcagctggcacgtcagctgtatgagctgctggttccgcaggcaattggtgcaaaaggtgatgcacagtttattgcccgtaaatttctgagtccgctggcagataaagatgcagttggtggtctgggtattgcaaaagcaggtaataaaccgcgttgggttcgtatgcgtgaagccggtgaacctggttgggaagaagaaaaagccaaagccgaagcacgtaaaagcaccgatcgtaccgcagatgttctgcgtgccctggcagattttggtctgaaaccgctgatgcgtgtttataccgatagcgatatgagcagcgttcagtggaaacctctgcgtaaaggtcaggcagttcgtacctgggatcgtgatatgtttcagcaggccattgaacgtatgatgagctgggaaagctggaatcagcgtgttggtgaagcctatgcaaaactggttgaacagaaaagccgtttcgagcagaaaaactttgttggtcaagaacacctggttcagctggtgaatcagctgcaacaggatatgaaagaagcaagccacggtctggaaagcaaagaacagaccgcacattatctgaccggtcgtgcactgcgtggtagcgataaagtttttgaaaaatgggaaaaactggatccggatgcaccgtttgatctgtatgataccgaaatcaaaaatgtgcagcgtcgtaatacccgtcgttttggtagccatgacctgtttgccaaactggcagaaccgaaatatcaggcactgtggcgtgaagatgcaagctttctgacccgttatgcagtgtataatagcattgtgcgcaaactgaatcacgccaaaatgtttgcaacctttacactgccggatgcaaccgcacatccgatttggacccgttttgataaattaggtggtaacctgcaccagtacacctttctgtttaatgaatttggtgaaggtcgtcatgccatccgttttcagaaactgctgaccgttgaagatggtgttgcaaaagaagttgacgacgttaccgttccgattagcatgagcgcacagctggatgatctgcttccgcgtgatccgcatgaactggttgcactgtattttcaggattatggtgcagaacagcatctggcaggtcgctttggtggtgccaaaattcagtatcgtcgcgatcagctgaatcatctgcatgcccgtcgtggtgcacgtgatgtttatctgaatctgagcgttcgtgttcagagccagagcgaagcccgtggtgaacgtcgccctccgtatgcagccgtttttcgtctggttggtgataatcatcgtgcctttgttcactttgataaactgagcgattatctggccgaacatcctgatgatggtaaactgggtagcgaaggtctgctgagcggtctgcgtgttatgagcgttgatctgggtctgcgtaccagcgcaagcattagcgtgtttcgtgttgcacgtaaagatgaactgaaaccgaatagcgaaggccgtgttccgttttgttttccgattgaaggtaatgaaaatctggttgcagtgcatgaacgtagtcagctgctgaaattaccgggtgaaacagaatcaaaagatctgcgtgcgattcgtgaagaacgtcagcgtaccctgcgtcagctgcgcacccagctggcatatctgcgtctgctggtgcgttgtggtagtgaagatgttggtcgtcgtgaacgtagctgggccaaactgatcgaacagccgatggatgcaaatcagatgacaccggattggcgtgaggcatttgaagatgagctgcagaaactgaaaagcctgtatggtatttgtggtgatcgtgaatggaccgaagccgtttatgaaagcgttcgtcgtgtttggcgtcacatgggtaaacaggttcgtgattggcgcaaagatgttcgtagtggcgaacgtccgaaaattcgtggttatcagaaagatgttgttggtggcaatagcattcgccagattgaatatctggaacgccagtacaaattcctgaaaagctggtcatttttcggtaaagttagcggtcaggttattcgtgccgaaaaaggtagccgttttgcaattacactgcgcgaacatattgatcatgccaaagaagatcgtctgaaaaagctggccgatcgcattattatggaagcactgggttatgtttatgccctggatgatgaacgtggtaaaggtaaatgggttgccaaatatccgccttgccagctgatcctgctggaagaactgagtgaatatcagtttaataacgatcgtccgcctagcgaaaataaccagctgatgcagtggtcccatcgtggtgtttttcaagaactgttaaatcaggcacaggttcacgatctgctggttggcaccatgtatgcagcatttagcagtcgttttgatgcacgtacaggtgcaccgggtattcgttgccgtcgtgttccggcacgttgtgcccgtgaacagaatccggaaccgtttccgtggtggctgaataaattcgttgcagaacataaactggatggttgtccgctgcgtgccgatgatctgatcccgaccggtgaaggtgaatttttcgttagcccgttttctgccgaagaaggtgattttcatcagattcatgcagatctgaatgcagcacagaatctgcaacgtcgtctgtggtcagattttgatatcagccagattcgtctgcgctgtgattggggtgaagttgatggcgaaccggtgctgattccgcgtaccaccggtaaacgtacagcagatagctatggtaacaaagtgttctataccaaaaccggtgtgacctattatgaacgtgaacgcggtaagaaacgtcgtaaagtgtttgcacaagaagaactgtcagaagaagaagccgaactgttagttgaagcagatgaagcgcgtgaaaaatcagttgttctgatgcgcgatccgagcggtattatcaatcgtggtgattggacacgtcagaaagaattttggagcatggttaatcagcgcattgaaggttatctggtgaaacaaattcgtagccgtgttcgtctgcaagaaagcgcatgtgaaaataccggtgatattgcaagcccgaaaaagaaacgtaaagttggtagcggtagtccggcagccaaaaagaagaaactggacggtagcggttcaaaacgtcctgcagcaaccaaaaaggcaggtcaggctaaaaagaaaaagtaa

SEQ ID NO: 85 - DNA, 3519 bp, synthetic construct
  misc_feature 1..3519: note = Ecoli Cas12b-M7
  source 1..3519: mol_type = other DNA
atgaagcggacggcggacgggagcgaatttgaaagcccgaaaaaaaaacgcaaagttgaaccgggcatggcagtgaaaagtatgaaagtgaaactgcgtctggataatatgccggaaattcgtgcaggcctgtggaaactgcataccgaagttaatgccggcgttcgctattataccgaatggctgagtctgctgcgtcaggaaaatctgtatcgtcgcagtccgaatggcgatggtgaacaggaatgctataaaaccgccgaagaatgcaaagccgaactgctggaacgtctgcgcgcccgccaggttgaaaatggtcattgcggtccggcaggtagcgatgatgaactgctgcagctggcacgccagctgtatgaactgctggttccgcaggcaattggtgccaaaggtgacgcccagtttattgcccgcaaatttctgagtccgctggccgataaagatgccgtgggtggcctgggtattgccaaagccggcaataagccgcgttgggttcgcatgcgtgaagccggcgaaccgggttgggaagaagaaaaagcaaaagccgaagcacgtaaaagcaccgatcgcaccgcagatgttctgcgtgcactggcagattttggtctgaaaccgctgatgcgtgtttataccgatagcgatatgagcagcgtgcagtggaaaccgctgcgcaaaggccaggccgtgcgcacatgggatcgtgatatgtttcagcaggccattgaacgtatgatgagttgggaaagttggaatcagcgtgtgggtgaagcctatgcaaaactggtggaacagaaaagtcgttttgaacagaaaaatttcgtgggtcaggaacatctggttcagctggtgaatcagctgcagcaggatatgaaagaagcaagccacggtctggaaagcaaagaacagaccgcacattatctgaccggccgtgccctgcgcggcagtgataaagtgtttgaaaaatgggaaaagctggaccctgatgcaccgtttgatctgtatgataccgaaattaagaacgtgcagcgccgtaatacccgccgctttggtagtcatgatctgtttgccaaactggcagaaccgaaatatcaggcactgtggcgcgaagatgccagttttctgacccgttatgccgtttataatagcattgtgcgcaaactgaatcatgccaaaatgtttgccacctttaccctgccggatgcaaccgcacatccgatttggacccgctttgataaactgggtggtaatctgcatcagtatacctttctgtttaatgaatttggtgagggccgtcatgcaattcgctttcagaaactgctgaccgtggaagatggcgtggcaaaagaagtggatgatgtgaccgtgccgattagcatgagcgcacagctggatgatctgctgccgcgtgatccgcatgaactggtggcactgtattttcaggattatggtgcagaacagcatctggccggccgttttggtggtgccaaaattcagtatcgccgtgatcagctgaatcatctgcatgcccgccgtggcgcccgtgatgtttatctgaatctgagcgttcgcgttcagagtcagagcgaagcacgtggtgaacgccgtccgccgtatgcagccgtgtttcgcctggttggcgataatcatcgcgcatttgtgcattttgataaattaagtgactacctggcagaacatccggatgatggtaaactgggtagtgaaggcctgctgagtggcctgcgtgttatgagtgtggatctgggcctgcgtaccagcgcaagtattagtgtgtttcgtgtggcacgtaaagatgaactgaaaccgaatagtgaaggccgcgttccgttttgttttccgattgaaggcaatgaaaatctggttgcagttcatgaacgcagccagctgctgaaactgccgggcgaaaccgaaagcaaagatctgcgcgcaattcgcgaagaacgtcagcgcaccctgcgtcagctgcgtacccagctggcctatctgcgcctgctggtgcgttgtggcagcgaagatgttggccgtcgtgaacgcagctgggcaaaactgattgaacagccgatggatgcaaatcagatgaccccggattggcgcgaagcatttgaagatgaactgcagaaactgaaaagtctgtatggcatttgtggtgaccgtgaatggaccgaagccgtgtatgaaagcgttcgccgcgtttggcgccacatgggcaaacaggttcgcgattggcgcaaagatgttcgtagcggcgaacgtccgaaaattcgtggttatcagaaagatgtggttggcggcaatagcattcgccagattgaatatctggaacgtcagtataaattcctgaaaagttggagctttttcggtaaagtgagtggtcaggttattcgtgccgaaaaaggtagtcgctttgcaattaccctgcgcgaacatattgatcatgccaaagaagatcgtctgaaaaaactggcagatcgtattattatggaagccctgggttatgtgtatgccctggatgatgaacgtggtaaaggcaaatgggtggcaaaatatccgccgtgccagctgattctgctggaagaactgagcgaatatcagtttaataatgatcgcccgccgagtgaaaataatcagctgatgcagtggagccatcgtggtgtgtttcaggaactgctgaatcaggcacaggttcatgatctgctggttggcaccatgtatgcagcctttagtagccgttttgatgcacgtaccggcgcaccgggtattcgttgtcgtcgcgttccggcccgctgcgctcgtgaacagaatccggaaccgtttccgtggtggctgaataagtttgtggccgaacataaactggatggttgtccgctgcgcgcagatgatctgattccgaccggtgaaggtgaatttttcgttagcccgtttagtgccgaagaaggtgactttcatcagattcatgccgatctgaatgccgcacagaatctgcagcgccgtctgtggagcgattttgatattagtcagattcgtctgcgttgtgattggggtgaagtggatggtgaaccggtgctgattccgcgtaccaccggtaaacgcaccgccgatagttatggcaataaggtgttttataccaaaaccggcgttacctattatgaacgtgaacgcggcaaaaaacgtcgcaaagtttttgcccaggaagaactgagtgaagaagaagccgaactgttagtggaagcagatgaagcacgtgaaaaaagcgtggtgctgatgcgcgatccgagtggtattattaatcgcggtgactggacccgtcagaaagaattttggagcatggttaatcagcgcattgaaggttatctggtgaaacagattcgtagccgtgttcgtctgcaggaaagtgcctgtgaaaataccggtgacattgcaagtaagcgcaccgcagatggaagcgaatttgaaagcccgaaaaaaaaaagaaaggtggaataa

SEQ ID NO: 86 - DNA, 3546 bp, synthetic construct
  misc_feature 1..3546: note = Ecoli Cas12b-M8
  source 1..3546: mol_type = other DNA
atgcccaagaagaagaggaaggttacgcgtatggccgtgaagagtatgaaggtgaagctgcggctggacaacatgcccgagatccgggccggcctgtggaagctgcacaccgaggtgaacgccggcgtgcggtactacaccgagtggctgagcctgctgcggcaggagaacctgtaccggcggagcccaaacggcgacggcgagcaggagtgctacaagaccgccgaggagtgcaaggccgagctgctggagcggctgcgggcccggcaggtggagaacggccactgcggccccgccggcagcgacgacgagctgctgcagctggcccggcagctgtacgagctgctggtgccccaggccatcggcgccaagggcgacgcccagttcatcgcccggaagttcctgagccccctggccgacaaggacgccgtgggcggcctgggcatcgccaaggccggcaacaagccccggtgggtgcggatgcgggaggccggcgagcccggctgggaggaggagaaggccaaggccgaggcccggaagagtaccgaccggaccgccgacgtgctgcgggccctggccgacttcggcctgaagcccctgatgcgggtgtacaccgacagcgacatgagcagcgtgcagtggaagccactgcggaagggccaggccgtgcggacctgggaccgggacatgttccagcaggccatcgagcggatgatgagctgggagagctggaaccagcgggtgggcgaggcctacgccaagctggtggagcagaagagtcggttcgagcagaagaacttcgtgggccaggagcacctggtgcagctggtgaaccagctgcagcaggacatgaaggaggccagccacggcctggagagcaaggagcagaccgcccactacctgaccggccgggccctgcggggcagcgacaaggtgttcgagaagtgggagaagctggaccccgacgcccccttcgacctgtacgacaccgagatcaagaacgtgcagcggcggaacacccggcggttcggcagccacgacctgttcgccaagctggccgagcccaagtaccaggccctgtggcgggaggacgccagcttcctgacccggtacgccgtgtacaacagcatcgtgcggaagctgaaccacgccaagatgttcgccaccttcaccctgcccgacgccaccgcccaccccatctggacccggttcgacaagctgggcggcaacctgcaccagtacaccttcctgttcaacgagttcggcgagggccggcacgccatccggttccagaagctgctgaccgtggaggacggcgtggccaaggaggtggacgacgtgaccgtgcccatcagcatgagcgcccagctggacgacctgctgccccgggacccccacgagctggtggccctgtacttccaggactacggcgccgagcagcacctggccggccggttcggcggcgccaagatccagtaccggcgggaccagctgaaccacctgcacgcccggcggggcgcccgggacgtgtacctgaacctgagcgtgcgggtgcagagccagagcgaggcccggggcgagcggcggccaccctacgccgccgtgttccggctggtgggcgacaaccaccgggccttcgtgcacttcgacaagctgagcgactacctggccgagcacccagacgacggcaagctgggcagcgagggcctgctgagcggcctgcgggtgatgagcgtggacctgggcctgcggaccagcgccagcatcagcgtgttccgggtggcccggaaggacgagctgaagcccaacagcgagggccgggtgcccttctgcttccccatcgagggcaacgagaacctggtggccgtgcacgagcggagccagctgctgaagctgcccggcgaaaccgagagcaaggacctgcgggccatccgggaggagcggcagcggaccctgcggcagctgcggacccagctggcctacctgcggctgctggtgcggtgcggcagcgaggacgtgggccggcgggagcggagctgggccaagctgatcgagcagcccatggacgccaaccagatgacccccgactggcgggaggccttcgaggacgagctgcagaagctgaagagtctgtacggcatctgcggcgaccgggagtggaccgaggccgtgtacgagagcgtgcggcgggtgtggcggcacatgggcaagcaggtgcgggactggcggaaggacgtgcggagcggcgagcggcccaagatccggggctaccagaaggacgtggtgggcggcaacagcatccggcagatcgagtacctggagcggcagtacaagttcctgaagagttggagcttcttcggcaaggtgagcggccaggtgatccgggccgagaagggcagccggttcgccatcaccctgcgggagcacatcgaccacgccaaggaggaccggctgaagaagctggccgaccggatcatcatggaggccctgggctacgtgtacgccctggacgacgagcggggcaagggcaagtgggtggccaagtacccaccctgccagctgatcctgctggaggagctgagcgagtaccagttcaacaacgaccggcccccaagcgagaacaaccagctgatgcagtggagccaccggggcgtgttccaggagctgctgaaccaggcccaggtgcacgacctgctggtgggcaccatgtacgccgccttcagcagccggttcgacgcccggaccggcgcccccggcatccggtgccggcgggtgcccgcccggtgcgcccgggagcagaacccagagcccttcccctggtggctgaacaagttcgtggccgagcacaagctggacggctgccccctgcgggccgacgacctgatccccaccggcgagggcgagttcttcgtgagccccttcagcgccgaggagggcgacttccaccagatccacgccgacctgaacgccgcccagaacctgcagcggcggctgtggagcgacttcgacatcagccagatccggctgcggtgcgactggggcgaggtggacggcgagcccgtgctgatcccccggaccaccggcaagcggaccgccgacagctacggcaacaaggtgttctacaccaagaccggcgtgacctactacgagcgggagcggggcaagaagcggcggaaggtgttcgcccaggaggagctgagcgaggaggaggccgagctgctggtggaggccgacgaggcccgggagaagagtgtggtgctgatgcgggaccccagcggcatcatcaaccggggcgactggacccggcagaaggagttctggagcatggtgaaccagcggatcgagggctacctggtgaagcagatccggagccgggtgcggctgcaggagagcgcctgcgagaacaccggcgacatcgctagcccaaagaagaagaggaaagtcggctctggcagccctgccgccaagaaaaagaagctggacggatctggcagcaagaggcctgctgccaccaagaaggccggccaggccaagaaaaaaaagtga

SEQ ID NO: 87 - DNA, 3240 bp, synthetic construct
  misc_feature 1..3240: note = Cas12i-M1 DNA
  source 1..3240: mol_type = other DNA
atgcatcatcatcatcaccatcccaagaagaagaggaaggttcccgggatgagcagcgccatcaagagctacaagagcgtgctgcgccccaacgagcgcaagaaccagctgctgaagagcaccatccagtgcctggaggacggcagcgccttcttcttcaagatgctgcagggcctgttcggcggcatcacccccgagatcgtgcgcttcagcaccgagcaggagaagcagcagcaggacatcgccctgtggtgcgccgtgaactggttccgccccgtgagccaggacagcctgacccacaccatcgccagcgacaacctggtggagaagttcgaggagtactacggcggcaccgccagcgacgccatcaagcagtacttcagcgccagcatcggcgagagctactactggaacgactgccgccagcagtactacgacctgtgccgcgagctgggcgtggaggtgagcgacctgacccacgacctggagatcctgtgccgcgagaagtgcctggccgtggccaccgagagcaaccagtacaacagcatcatcagcgtgctgttcggcaccggcagaaaggaggaccgcagcgtgaagctgcgcatcaccaagaagatcctggaggccatcagcaacctgaaggagatccccaagaacgtggcccccatccaggagatcatcctgaacgtggccaaggccaccaaggagaccttccgccaggtgtacgccggcaacctgggcgcccccagcaccctggagagattcatcgccaaggacggccagaaggagttcgacctgaagaagctgcagaccgacctgaagaaggtgatccgcggcaagagcaaggagcgcgactggtgctgccaggaggagctgcgcagctacgtggagcagaacaccatccagtacgacctgtgggcctggggcgagatgttcaacaaggcccacaccgccctgaagatcaagagcacccgcaactacaacttcgccaagcagcgcctggagcagttcaagagaatccagagcctgaacaacctgctggtggtgaagaagctgaacgacttcttcgacagcgagttcttcagcggcgaggagacctacaccatctgcgtgcaccacctgggcggcaagagactgagcaagctgtacaaggcctgggaggacgaccccgccgaccccgagaacgccatcgtggtgctgtgcgacgacctgaagaacaacttcaaggccgagcccatccgcaacatcctgcgctacatcttcaccatccgccaggagtgcagcgcccaggacatcctggccgccgccaagtacaaccagcagctggaccgctacaagagccagaaggccaaccccagcgtgctgggcaaccagggcttcacctggagaaacgccgtgatcctgcccgagaaggcccagcgcaacgaccgccccaacagcctggacctgcgcatctggctgtacctgaagctgcgccaccccgacggccgctggaagaagcaccacatccccttctacgacacccgcttcttccaggagatctacgccgccggcaacagccccgtggacacctgccagttccgcaccccccgcttcggctaccacctgcccaagctgaccgaccagaccgccatccgcgtgaacaagaagcacgtgaaggccgccaagaccgaggcccgcatccgcctggccatccagcagggcaccctgcccgtgagcaacctgaagatcaccagaatcagcgccaccatcaacagcaagggccaggtgcgcatccccgtgaagttcgacgtgggccgccagaagggcaccctgcagatcggcgaccgcttctgcggctacgaccagaaccagaccgccagccacgcctacagcctgtgggaggtggtgaaggagggccagtaccacaaggagctgggctgcttcgtgcgcttcatcagcagcggcgacatcgtgagcatcaccgagaaccgcggcaaccagttcgaccagctgagctacgagggcctggcctacccccagtacgccgactggcgcaagaaggccagcaagttcgtgagcctgtggcagatcaccaagaagaacaagaagaaggagatcgtgaccgtggaggccaaggagaagttcgacgccatctgcaagtaccagccccgcctgtacaagttcaacaaggagtacgcctacctgctgcgcgacatcgtgcgcggcaagagcctggtggagctgcagcagatccgccaggagatcttccgcttcatcgagcaggactgcggcgtgacccgcctgggcagcctgagcctgagcaccctggagaccgtgaaggccgtgaagggcatcatctacagctacttcagcaccgccctgaacgccagcaagaacaaccccatcagcgacgagcagcgcaaggagttcgaccccgagctgttcgccctgctggagaagctggagctgatccgcacccgcaagaagaagcagaaggtggagcgcatcgccaacagcctgatccagacctgcctggagaacaacatcaagttcatccgcggcgagggcgacctgagcaccaccaacaacgccaccaagaagaaggccaacagccgcagcatggactggctggcccgcggcgtgttcaacaagatccgccagctggcccccatgcacaacatcaccctgttcggctgcggcagcctgtacaccagccaccaggaccccctggtgcaccgcaaccccgacaaggccatgaagtgccgctgggccgccatccccgtgaaggacatcggcgactgggtgctgcgcaagctgagccagaacctgcgcgccaagaacatcggcaccggcgagtactaccaccagggcgtgaaggagttcctgagccactacgagctgcaggacctggaggaggagctgctgaagtggcgcagcgaccgcaagagcaacatcccctgctgggtgctgcagaaccgcctggccgagaagctgggcaacaaggaggccgtggtgtacatccccgtgcgcggcggccgcatctacttcgccacccacaaggtggccaccggcgccgtgagcatcgtgttcgaccagaagcaggtgtgggtgtgcaacgccgaccacgtggccgccgccaacatcgccctgaccgtgaagggcatcggcgagcagagcagcgacgaggagaaccccgacggcagccgcatcaagctgcagctgaccagcgctagcccaaagaagaagaggaaagtctag

SEQ ID NO: 88 - DNA, 3240 bp, synthetic construct
  misc_feature 1..3240: note = Cas12i-M2 DNA
  source 1..3240: mol_type = other DNA
atgcatcatcatcatcaccatcccaagaagaagaggaaggttcccgggatgagcagcgccatcaagagctacaagagcgtgctgcgccccaacgagcgcaagaaccagctgctgaagagcaccatccagtgcctggaggacggcagcgccttcttcttcaagatgctgcagggcctgttcggcggcatcacccccgagatcgtgcgcttcagcaccgagcaggagaagcagcagcaggacatcgccctgtggtgcgccgtgaactggttccgccccgtgagccaggacagcctgacccacaccatcgccagcgacaacctggtggagaagttcgaggagtactacggcggcaccgccagcgacgccatcaagcagtacttcagcgccagcatcggcgagagctactactggaacgactgccgccagcagtactacgacctgtgccgcgagctgggcgtggaggtgagcgacctgacccacgacctggagatcctgtgccgcgagaagtgcctggccgtggccaccgagagcaaccagtacaacagcatcatcagcgtgctgttcggcaccggcagaaaggaggaccgcagcgtgaagctgcgcatcaccaagaagatcctggaggccatcagcaacctgaaggagatccccaagaacgtggcccccatccaggagatcatcctgaacgtggccaaggccaccaaggagaccttccgccaggtgtacgccggcaacctgggcgcccccagcaccctggagagattcatcgccaaggacggccagaaggagttcgacctgaagaagctgcagaccgacctgaagaaggtgatccgcggcaagagcaaggagcgcgactggtgctgccaggaggagctgcgcagctacgtggagcagaacaccatccagtacgacctgtgggcctggggcgagatgttcaacaaggcccacaccgccctgaagatcaagagcacccgcaactacaacttcgccaagcagcgcctggagcagttcaagagaatccagagcctgaacaacctgctggtggtgaagaagctgaacgacttcttcgacagcgagttcttcagcggcgaggagacctacaccatctgcgtgcaccacctgggcggcaagagactgagcaagctgtacaaggcctgggaggacgaccccgccgaccccgagaacgccatcgtggtgctgtgcgacgacctgaagaacaacttcaagaaggagcccatccgcaacatcctgcgctacatcttcaccatccgccaggagtgcagcgcccaggacatcctggccgccgccaagtacaaccagcagctggaccgctacaagagccagaaggccaaccccagcgtgctgggcaaccagggcttcacctggagaaacgccgtgatcctgcccgagaaggcccagcgcaacgaccgccccaacagcctggacctgcgcatctggctgtacctgaagctgcgccaccccgacggccgctggaagaagcaccacatccccttctacgacacccgcttcttccaggagatctacgccgccggcaacagccccgtggacacctgccagttccgcaccccccgcttcggctaccacctgcccaagctgaccgaccagaccgccatccgcgtgaacaagaagcacgtgaaggccgccaagaccgaggcccgcatccgcctggccatccagcagggcaccctgcccgtgagcaacctgaagatcaccagaatcagcgccaccatcaacagcaagggccaggtgcgcatccccgtgaagttcgacgtgggccgccagaagggcaccctgcagatcggcgaccgcttctgcggctacgaccagaaccagaccgccagccacgcctacagcctgtgggaggtggtgaaggagggccagtaccacaaggagctgggctgcttcgtgcgcttcatcagcagcggcgacatcgtgagcatcaccgagaaccgcggcaaccagttcgaccagctgagctacgagggcctggcctacccccagtacgccgactggcgcaagaaggccagcaagttcgtgagcctgtggcagatcaccaagaagaacaagaagaaggagatcgtgaccgtggaggccaaggagaagttcgacgccatctgcaagtaccagccccgcctgtacaagttcaacaaggagtacgcctacctgctgcgcgacatcgtgcgcggcaagagcctggtggagctgcagcagatccgccaggagatcttccgcttcatcgagcaggactgcggcgtgacccgcctgggcagcctgagcctgagcaccctggagaccgtgaaggccgtgaagggcatcatctacagctacttcagcaccgccctgaacgccagcaagaacaaccccatcagcgacgagcagcgcaaggagttcgaccccgagctgttcgccctgctggagaagctggagctgatccgcacccgcaagaagaagcagaaggtggagcgcatcgccaacagcctgatccagacctgcctggagaacaacatcaagttcatccgcggcgagggcgacctgagcaccaccaacaacgccaccaagaagaaggccaacagccgcagcatggactggctggcccgcggcgtgttcaacaagatccgccagctggcccccatgcacaacatcaccctgttcggctgcggcagcctgtacaccagccaccaggaccccctggtgcaccgcaaccccgacaaggccatgaagtgccgctgggccgccatccccgtgaaggacatcggcgactgggtgctgcgcaagctgagccagaacctgcgcgccaagaacatcggcaccggcgagtactaccaccagggcgtgaaggagttcctgagccactacgagctgcaggacctggaggaggagctgctgaagtggcgcagcgaccgcaagagcaacatcccctgctgggtgctgcagaaccgcctggccgagaagctgggcaacaaggaggccgtggtgtacatccccgtgcgcggcggccgcatctacttcgccacccacaaggtggccaccggcgccgtgagcatcgtgttcgaccagaagcaggtgtgggtgtgcaacgccgaccacgtggccgccgccaacatcgccctgaccgtgaagggcatcggcgagcagagcagcgacgaggagaaccccgacggcagccgcatcaagctgcagctgaccagcgctagcccaaagaagaagaggaaagtctag

SEQ ID NO: 89 - DNA, 3216 bp, synthetic construct
  misc_feature 1..3216: note = Cas12i-M3 DNA
  source 1..3216: mol_type = other DNA
cccaagaagaagaggaaggttcccgggatgagcagcgccatcaagagctacaagagcgtgctgcgccccaacgagcgcaagaaccagctgctgaagagcaccatccagtgcctggaggacggcagcgccttcttcttcaagatgctgcagggcctgttcggcggcatcacccccgagatcgtgcgcttcagcaccgagcaggagaagcagcagcaggacatcgccctgtggtgcgccgtgaactggttccgccccgtgagccaggacagcctgacccacaccatcgccagcgacaacctggtggagaagttcgaggagtactacggcggcaccgccagcgacgccatcaagcagtacttcagcgccagcatcggcgagagctactactggaacgactgccgccagcagtactacgacctgtgccgcgagctgggcgtggaggtgagcgacctgacccacgacctggagatcctgtgccgcgagaagtgcctggccgtggccaccgagagcaaccagtacaacagcatcatcagcgtgctgttcggcaccggcagaaaggaggaccgcagcgtgaagctgcgcatcaccaagaagatcctggaggccatcagcaacctgaaggagatccccaagaacgtggcccccatccaggagatcatcctgaacgtggccaaggccaccaaggagaccttccgccaggtgtacgccggcaacctgggcgcccccagcaccctggagagattcatcgccaaggacggccagaaggagttcgacctgaagaagctgcagaccgacctgaagaaggtgatccgcggcaagagcaaggagcgcgactggtgctgccaggaggagctgcgcagctacgtggagcagaacaccatccagtacgacctgtgggcctggggcgagatgttcaacaaggcccacaccgccctgaagatcaagagcacccgcaactacaacttcgccaagcagcgcctggagcagttcaagagaatccagagcctgaacaacctgctggtggtgaagaagctgaacgacttcttcgacagcgagttcttcagcggcgaggagacctacaccatctgcgtgcaccacctgggcggcaagagactgagcaagctgtacaaggcctgggaggacgaccccgccgaccccgagaacgccatcgtggtgctgtgcgacgacctgaagaacaacttcaagaaggagcccatccgcaacatcctgcgctacatcttcaccatccgccaggagtgcagcgcccaggacatcctggccgccgccaagtacaaccagcagctggaccgctacaagagccagaaggccaaccccagcgtgctgggcaaccagggcttcacctggagaaacgccgtgatcctgcccgagaaggcccagcgcaacgaccgccccaacagcctggacctgcgcatctggctgtacctgaagctgcgccaccccgacggccgctggaagaagcaccacatccccttctacgacacccgcttcttccaggagatctacgccgccggcaacagccccgtggacacctgccagttccgcaccccccgcttcggctaccacctgcccaagctgaccgaccagaccgccatccgcgtgaacaagaagcacgtgaaggccgccaagaccgaggcccgcatccgcctggccatccagcagggcaccctgcccgtgagcaacctgaagatcaccagaatcagcgccaccatcaacagcaagggccaggtgcgcatccccgtgaagttcgacgtgggccgccagaagggcaccctgcagatcggcgaccgcttctgcggctacgaccagaaccagaccgccagccacgcctacagcctgtgggaggtggtgaaggagggccagtaccacaaggagctgggctgcttcgtgcgcttcatcagcagcggcgacatcgtgagcatcaccgagaaccgcggcaaccagttcgaccagctgagctacgagggcctggcctacccccagtacgccgactggcgcaagaaggccagcaagttcgtgagcctgtggcagatcaccaagaagaacaagaagaaggagatcgtgaccgtggaggccaaggagaagttcgacgccatctgcaagtaccagccccgcctgtacaagttcaacaaggagtacgcctacctgctgcgcgacatcgtgcgcggcaagagcctggtggagctgcagcagatccgccaggagatcttccgcttcatcgagcaggactgcggcgtgacccgcctgggcagcctgagcctgagcaccctggagaccgtgaaggccgtgaagggcatcatctacagctacttcagcaccgccctgaacgccagcaagaacaaccccatcagcgacgagcagcgcaaggagttcgaccccgagctgttcgccctgctggagaagctggagctgatccgcacccgcaagaagaagcagaaggtggagcgcatcgccaacagcctgatccagacctgcctggagaacaacatcaagttcatccgcggcgagggcgacctgagcaccaccaacaacgccaccaagaagaaggccaacagccgcagcatggactggctggcccgcggcgtgttcaacaagatccgccagctggcccccatgcacaacatcaccctgttcggctgcggcagcctgtacaccagccaccaggaccccctggtgcaccgcaaccccgacaaggccatgaagtgccgctgggccgccatccccgtgaaggacatcggcgactgggtgctgcgcaagctgagccagaacctgcgcgccaagaacatcggcaccggcgagtactaccaccagggcgtgaaggagttcctgagccactacgagctgcaggacctggaggaggagctgctgaagtggcgcagcgaccgcaagagcaacatcccctgctgggtgctgcagaaccgcctggccgagaagctgggcaacaaggaggccgtggtgtacatccccgtgcgcggcggccgcatctacttcgccacccacaaggtggccaccggcgccgtgagcatcgtgttcgaccagaagcaggtgtgggtgtgcaacgccgaccacgtggccgccgccaacatcgccctgaccgtgaagggcatcggcgagcagagcagcgacgaggagaaccccgacggcagccgcatcaagctgcagctgaccagcgctagcccaaagaagaagaggaaagtc

SEQ ID NO: 90 - RNA, 113 nt, synthetic construct
  modified_base 3: mod_base = OTHER; note = thymine
  modified_base 6: mod_base = OTHER; note = thymine
  modified_base 8: mod_base = OTHER; note = thymine
  modified_base 10: mod_base = OTHER; note = thymine
  modified_base 22..26: mod_base = OTHER; note = thymine
  modified_base 34: mod_base = OTHER; note = thymine
  modified_base 36: mod_base = OTHER; note = thymine
  modified_base 42: mod_base = OTHER; note = thymine
  modified_base 49..51: mod_base = OTHER; note = thymine
  modified_base 57: mod_base = OTHER; note = thymine
  modified_base 69..70: mod_base = OTHER; note = thymine
  modified_base 75..76: mod_base = OTHER; note = thymine
  modified_base 85: mod_base = OTHER; note = thymine
  modified_base 94: mod_base = OTHER; note = thymine
  modified_base 97: mod_base = OTHER; note = thymine
  modified_base 99: mod_base = OTHER; note = thymine
  misc_feature 1..113: note = 12b-gRNA1-3ex(113)
  source 1..113: mol_type = other RNA
  modified_base 1..3: mod_base = OTHER; note = 2'-O-methyl nucleotide
  modified_base 1..4: mod_base = OTHER; note = phosphorothioate internucleotide linkage
  modified_base 111..113: mod_base = OTHER; note = 2'-O-methyl nucleotide
  modified_base 110..113: mod_base = OTHER; note = phosphorothioate internucleotide linkage
ggtcgtctataggacggcgagtttttcaacgggtgtgccaatggccactttccaggtggcaaagcccgttgagcttcaaagaagtggcacagatagtgtggggaaggggcccc

SEQ ID NO: 91 - protein, 1129 aa, synthetic construct
  REGION 1..1129: note = wt AaCas12b
MAVKSMKVKLRLDNMPEIRAGLWKLHTEVNAGVRYYTEWLSLLRQENLYRRSPNGDGEQECYKTAEECKAELLERLRARQVENGHCGPAGSDDELLQLARQLYELLVPQAIGAKGDAQQIARKFLSPLADKDAVGGLGIAKAGNKPRWVRMREAGEPGWEEEKAKAEARKSTDRTADVLRALADFGLKPLMRVYTDSDMSSVQWKPLRKGQAVRTWDRDMFQQAIERMMSWESWNQRVGEAYAKLVEQKSRFEQKNFVGQEHLVQLVNQLQQDMKEASHGLESKEQTAHYLTGRALRGSDKVFEKWEKLDPDAPFDLYDTEIKNVQRRNTRREGSHDLFAKLAEPKYQALWREDASFLTRYAVYNSIVRKLNHAKMFATFTLPDATAHPIWTREDKLGGNLHQYTFLENEFGEGRHAIRFQKLLTVEDGVAKEVDDVTVPISMSAQLDDLLPRDPHELVALYFQDYGAEQHLAGEFGGAKIQYRRDQLNHLHARRGARDVYLNLSVRVQSQSEARGERRPPYAAVFRLVGDNHRAFVHFDKLSDYLAEHPDDGKLGSEGLLSGLRVMSVDLGLRTSASISVFRVARKDELKPNSEGRVPFCFPIEGNENLVAVHERSQLLKLPGETESKDLRAIREERQRTLRQLRTQLAYLRLLVRCGSEDVGRRERSWAKLIEQPMDANQMTPDWREAFEDELQKLKSLYGICGDREWTEAVYESVRRVWRHMGKQVRDWRKDVRSGERPKIRGYQKDVVGGNSIEQIEYLERQYKFLKSWSFFGKVSGQVIRAEKGSRFAITLREHIDHAKEDRLKKLADRIIMEALGYVYALDDERGKGKWVAKYPPCQLILLEELSEYQFNNDRPPSENNQLMQWSHRGVFQELLNQAQVHDLLVGTMYAAFSSREDARTGAPGIRCRRVPARCAREQNPEPFPWWLNKFVAEHKLDGCPLRADDLIPTGEGEFFVSPFSAEEGDFHQIHADLNAAQNLQRRLWSDFDISQIRLRCDWGEVDGEPVLIPRTTGKRTADSYGNKVFYTKTGVTYYERERGKKRRKVFAQEELSEEEAELLVEADEAREKSVVLMRDPSGIINRGDWTRQKEFWSMVNQRIEGYLVKQIRSRVRLQESACENTGDI

SEQ ID NO: 92 - protein, 1054 aa, synthetic construct
  REGION 1..1054: note = wt Cas12i2
MSSAIKSYKSVLRPNERKNQLLKSTIQCLEDGSAFFFKMLQGLFGGITPEIVRFSTEQEKQQQDIALWCAVNWFRPVSQDSLTHTIASDNLVEKFEEYYGGTASDAIKQYFSASIGESYYWNDCRQQYYDLCRELGVEVSDLTHDLEILCREKCLAVATESNQNNSIISVLFGTGEKEDRSVKLRITKKILEAISNLKEIPKNVAPIQEIILNVAKATKETFRQVYAGNLGAPSTLEKFIAKDGQKEFDLKKLQTDLKKVIRGKSKERDWCCQEELRSYVEQNTIQYDLWAWGEMFNKAHTALKIKSTRNYNFAKQRLEQFKEIQSLNNLLVVKKLNDFFDSEFFSGEETYTICVHHLGGKDLSKLYKAWEDDPADPENAIVVLCDDLKNNFKKEPIRNILRYIFTIRQECSAQDILAAAKYNQQLDRYKSQKANPSVLGNQGFTWTNAVILPEKAQRNDRPNSLDLRIWLYLKLRHPDGRWKKHHIPFYDTRFFQEIYAAGNSPVDTCQFRTPRFGYHLPKLTDQTAIRVNKKHVKAAKTEARIRLAIQQGTLPVSNLKITEISATINSKGQVRIPVKFDVGRQKGTLQIGDRFCGYDQNQTASHAYSLWEVVKEGQYHKELGCFVRFISSGDIVSITENRGNQFDQLSYEGLAYPQYADWRKKASKFVSLWQITKKNKKKEIVTVEAKEKFDAICKYQPRLYKFNKEYAYLLRDIVRGKSLVELQQIRQEIFRFIEQDCGVTRLGSLSLSTLETVKAVKGIIYSYFSTALNASKNNPISDEQRKEFDPELFALLEKLELIRTRKKKQKVERIANSLIQTCLENNIKFIRGEGDLSTTNNATKKKANSRSMDWLARGVFNKIRQLAPMHNITLFGCGSLYTSHQDPLVHRNPDKAMKCRWAAIPVKDIGDWVLRKLSQNLRAKNIGTGEYYHQGVKEFLSHYELQDLEEELLKWRSDRKSNIPCWVLQNRLAEKLGNKEAVVYIPVRGGRIYFATHKVATGAVSIVFDQKQVWVCNADHVAAANIALTVKGIGEQSSDEENPDGSRIKLQLTS